European Patent Application EP 4 644 556 A1, published November 5, 2025. Title: Method for production of adeno-associated virus and set of vectors for production of adeno-associated virus. Applicant: FUJIFILM Corporation. The sequence listing filed with the application follows.

SEQUENCE LISTING (10 sequences)

SEQ ID NO: 1 - DNA, 6073 bp, synthetic construct
  misc_feature 1..6073: note = plasmid
  source 1..6073: mol_type = other DNA
gatccacgggtggcatccctgtgacccctccccagtgcctctcctggccctggaagttgccactccagtgcccaccagccttgtcctaataaaattaagttgcatcattttgtctgactaggtgtccttctataatattatggggtggaggggggtggtatggagcaaggggcaagttgggaagacaacctgtagggcctgcggggtctattgggaaccaagctggagtgcagtggcacaatcttggctcactgcaatctccgcctcctgggttcaagcgattctcctgcctcagcctcccgagttgttgggattccaggcatgcatgaccaggctcagctaatttttgtttttttggtagagacggggtttcaccatattggccaggctggtctccaactcctaatctcaggtgatctacccaccttggcctcccaaattgctgggattacaggcgtgaaccactgctcccttccctgtccttatcgatagatctaggaacccctagtgatggagttggccactccctctctgcgcgctcgctcgctcactgaggccgggcgaccaaaggtcgcccgacgcccgggctttgcccgggcggcctcagtgagcgagcgagcgcgcagctgcctgcaggcagcttggcactggccgtcgttttacaacgtcgtgactgggaaaaccctggcgttacccaacttaatcgccttgcagcacatccccctttcgccagctggcgtaatagcgaagaggcccgcaccgatcgcccttcccaacagttgcgcagcctgaatggcgaatggcgcctgatgcggtattttctccttacgcatctgtgcggtatttcacaccgcatacgtcaaagcaaccatagtacgcgccctgtagcggcgcattaagcgcggcgggtgtggtggttacgcgcagcgtgaccgctacacttgccagcgccctagcgcccgctcctttcgctttcttcccttcctttctcgccacgttcgccggctttccccgtcaagctctaaatcgggggctccctttagggttccgatttagtgctttacggcacctcgaccccaaaaaacttgatttgggtgatggttcacgtagtgggccatcgccctgatagacggtttttcgccctttgacgttggagtccacgttctttaatagtggactcttgttccaaactggaacaacactcaaccctatctcgggctattcttttgatttataagggattttgccgatttcggcctattggttaaaaaatgagctgatttaacaaaaatttaacgcgaattttaacaaaatattaacgtttacaattttatggtgcactctcagtacaatctgctctgatgccgcatagttaagccagccccgacacccgccaacacccgctgacgcgccctgacgggcttgtctgctcccggcatccgcttacagacaagctgtgaccgtctccgggagctgcatgtgtcagaggttttcaccgtcatcaccgaaacgcgcgagacgaaagggcctcgtgatacgcctatttttataggttaatgtcatgataataatggtttcttagacgtcaggtggcacttttcggggaaatgtgcgcggaacccctatttgtttatttttctaaatacattcaaatatgtatccgctcatgagacaataaccctgataaatgcttcaataatattgaaaaaggaagagtatgagtattcaacatttccgtgtcgcccttattcccttttttgcggcattttgccttcctgtttttgctcacccagaaacgctggtgaaagtaaaagatgctgaagatcagttgggtgcacgagtgggttacatcgaactggatctcaacagcggtaagatccttgagagttttcgccccgaagaacgttttccaatgatgagcacttttaaagttctgctatgtggcgcggtattatcccgtattgacgccgggcaagagcaactcggtcgccgcatacactattctcagaatgacttggttgagtactcaccagtcacagaaaagcatcttacggatggcatgacagtaagagaattatgcagtgctgccataaccatgagtgataacactgcggccaacttacttctgacaacgatcggaggaccgaaggagctaaccgcttttttgcacaacatgggggatcatgtaactcgccttgatcgttgggaaccggagctgaatgaagccataccaaacgacgagcgtgacaccacgatgcctgtagcaatggcaacaacgttgcgcaaactattaactggcgaactacttactctagcttcccggcaacaattaatagactggatggaggcggataaagttgcaggaccacttctgcgctcggcccttccggctggctggtttattgctgataaatctggagccggtgagcgtgggtctcgcggtatcattgcagcactggggccagatggtaagccctcccgtatcgtagttatctacacgacggggagtcaggcaactatggatgaacgaaatagacagatcgctgagataggtgcctcactgattaagcattggtaactgtcagaccaagtttactcatatatactttagattgatttaaaacttcatttttaatttaaaaggatctaggtgaagatcctttttgataatctcatgaccaaaatcccttaacgtgagttttcgttccactgagcgtcagaccccgtagaaaagatcaaaggatcttcttgagatcctttttttctgcgcgtaatctgctgcttgcaaacaaaaaaaccaccgctaccagcggtggtttgtttgccggatcaagagctaccaactctttttccgaaggtaactggcttcagcagagcgcagataccaaatactgttcttctagtgtagccgtagttaggccaccacttcaagaactctgtagcaccgcctacatacctcgctctgctaatcctgttaccagtggctgctgccagtggcgataagtcgtgtcttaccgggttggactcaagacgatagttaccggataaggcgcagcggtcgggctgaacggggggttcgtgcacacagcccagcttggagcgaacgacctacaccgaactgagatacctacagcgtgagctatgagaaagcgccacgcttcccgaagggagaaaggcggacaggtatccggtaagcggcagggtcggaacaggagagcgcacgagggagcttccagggggaaacgcctggtatctttatagtcctgtcgggtttcgccacctctgacttgagcgtcgatttttgtgatgctcgtcaggggggcggagcctatggaaaaacgccagcaacgcggcctttttacggttcctggccttttgctggccttttgctcacatgttctttcctgcgttatcccctgattctgtggataaccgtattaccgcctttgagtgagctgataccgctcgccgcagccgaacgaccgagcgcagcgagtcagtgagcgaggaagcggaagagcgcccaatacgcaaaccgcctctccccgcgcgttggccgattcattaatgcagctggcacgacaggtttcccgactggaaagcgggcagtgagcgcaacgcaattaatgtgagttagctcactcattaggcaccccaggctttacactttatgcttccggctcgtatgttgtgtggaattgtgagcggataacaatttcacacaggaaacagctatgaccatgattacgaattgcctgcaggcagctgcgcgctcgctcgctcactgaggccgcccgggcaaagcccgggcgtcgggcgacctttggtcgcccggcctcagtgagcgagcgagcgcgcagagagggagtggccaactccatcactaggggttcctatcgatatcaagctttaatagtaatcaattacggggtcattagttcatagcccatatatggagttccgcgttacataacttacggtaaatggcccgcctggctgaccgcccaacgacccccgcccattgacgtcaataatgacgtatgttcccatagtaacgccaatagggactttccattgacgtcaatgggtggagtatttacggtaaactgcccacttggcagtacatcaagtgtatcatatgccaagtacgccccctattgacgtcaatgacggtaaatggcccgcctggcattatgcccagtacatgaccttatgggactttcctacttggcagtacatctacgtattagtcatcgctattaccatggtgatgcggttttggcagtacatcaatgggcgtggatagcggtttgactcacggggatttccaagtctccaccccattgacgtcaatgggagtttgttttggcaccaaaatcaacgggactttccaaaatgtcgtaacaactccgccccattgacgcaaatgggcggtaggcgtgtacggtgggaggtctatataagcagagctggtttagtggatatccttaagggcccagccggcctcgcgagaattctctagcaagctgtgaccggcgcctacgctagacgccaccatggagagcgacgagagcggcctgcccgccatggagatcgagtgccgcatcaccggcaccctgaacggcgtggagttcgagctggtgggcggcggagagggcacccccaagcagggccgcatgaccaacaagatgaagagcaccaaaggcgccctgaccttcagcccctacctgctgagccacgtgatgggctacggcttctaccacttcggcacctaccccagcggctacgagaaccccttcctgcacgccatcaacaacggcggctacaccaacacccgcatcgagaagtacgaggacggcggcgtgctgcacgtgagcttcagctaccgctacgaggccggccgcgtgatcggcgacttcaaggtggtgggcaccggcttccccgaggacagcgtgatcttcaccgacaagatcatccgcagcaacgccaccgtggagcacctgcaccccatgggcgataacgtgctggtgggcagcttcgcccgcaccttcagcctgcgcgacggcggctactacagcttcgtggtggacagccacatgcacttcaagagcgccatccaccccagcatcctgcagaacgggggccccatgttcgccttccgccgcgtggaggagctgcacagcaacaccgagctgggcatcgtggagtaccagcacgccttcaagacccccatcgccttcgccagatcccgcgctcagtcgtccaattctgccgtggacggcaccgccggacccggctccaccggatctcgcgagggcagaggaagtcttctaacatgcggtgacgtggaggagaatcccggccctatgaccgagtacaagcccacggtgcgcctcgccacccgcgacgacgtccccagggccgtacgcaccctcgccgccgcgttcgccgactaccccgccacgcgccacaccgtcgatccggaccgccacatcgagcgggtcaccgagctgcaagaactcttcctcacgcgcgtcgggctcgacatcggcaaggtgtgggtcgcggacgacggcgccgcggtggcggtctggaccacgccggagagcgtcgaagcgggggcggtgttcgccgagatcggcccgcgcatggccgagttgagcggttcccggctggccgcgcagcaacagatggaaggcctcctggcgccgcaccggcccaaggagcccgcgtggttcctggccaccgtcggcgtctcgcccgaccaccagggcaagggtctgggcagcgccgtcgtgctccccggagtggaggcggccgagcgcgccggggtgcccgccttcctggagacctccgcgccccgcaacctccccttctacgagcggctcggcttcaccgtcaccgccgacgtcgaggtgcccgaaggaccgcgcacctggtgcatgacccgcaagcccggtgcctgaaatcaacctctggattacaaaatttgtgaaagattgactggtattcttaactatgttgctccttttacgctatgtggatacgctgctttaatgcctttgtatcagtt

SEQ ID NO: 2 - DNA, 11956 bp, synthetic construct
  misc_feature 1..11956: note = plasmid
  source 1..11956: mol_type = other DNA
atgactctcttaaggtagccaaatttccataggctccgcccccctgacgagcatcacaaaaatcgacgctcaagtcagaggtggcgaaacccgacaggactataaagataccaggcgtttccccctggaagctccctcgtgcgctctcctgttccgaccctgccgcttaccggatacctgtccgcctttctcccttcgggaagcgtggcgctttctcatagctcacgctgtaggtatctcagttcggtgtaggtcgttcgctccaagctgggctgtgtgcacgaaccccccgttcagcccgaccgctgcgccttatccggtaactatcgtcttgagtccaacccggtaagacacgacttatcgccactggcagcagccactggtaacaggattagcagagcgaggtatgtaggcggtgctacagagttcttgaagtggtggcctaactacggctacactagaaggacagtatttggtatctgcgctctgctgaagccagttaccttcggaaaaagagttggtagctcttgatccggcaaacaaaccaccgctggtagcggtggtttttttgtttgcaagcagcagattacgcgcagaaaaaaaggatctcaagaagatcctttgatcttttctacggggtctgacgctcagtggaacgaaaactcacgttaagggattttggtcatgagattatcaaaaaggatcttcacctagatccttttaaattaaaaatgaagttttaaatcaatctaaagtatatatgagtaaacttggtctgacagttaccaatgcttaatcagtgaggcacctatctcagcgatctgtctatttcgttcatccatagttgcctgactccccgtcgtgtagataactacgatacgggagggcttaccatctggccccagtgctgcaatgataccgcgagacccacgctcaccggctccagatttatcagcaataaaccagccagccggaagggccgagcgcagaagtggtcctgcaactttatccgcctccatccagtctattaattgttgccgggaagctagagtaagtagttcgccagttaatagtttgcgcaacgttgttgccattgctacaggcatcgtggtgtcacgctcgtcgtttggtatggcttcattcagctccggttcccaacgatcaaggcgagttacatgatcccccatgttgtgcaaaaaagcggttagctccttcggtcctccgatcgttgtcagaagtaagttggccgcagtgttatcactcatggttatggcagcactgcataattctcttactgtcatgccatccgtaagatgcttttctgtgactggtgagtactcaaccaagtcattctgagaatagtgtatgcggcgaccgagttgctcttgcccggcgtcaatacgggataataccgcgccacatagcagaactttaaaagtgctcatcattggaaaacgttcttcggggcgaaaactctcaaggatcttaccgctgttgagatccagttcgatgtaacccactcgtgcacccaactgatcttcagcatcttttactttcaccagcgtttctgggtgagcaaaaacaggaaggcaaaatgccgcaaaaaagggaataagggcgacacggaaatgttgaatactcatactcttcctttttcaatattattgaagcatttatcagggttattgtctcatgagcggatacatatttgaatgtatttagaaaaataaacaaataggggttccgcgcacatttccccgaaaagtgccacctaaattgtaagcgttaatattttgttaaaattcgcgttaaatttttgttaaatcagctcattttttaaccaataggccgaaatcggcaaaatcccttataaatcaaaagaatagaccgagatagggttgagtgttgttccagtttggaacaagagtccactattaaagaacgtggactccaacgtcaaagggcgaaaaaccgtctatcagggcgatggcccactacgtgaaccatcaccctaatcaagttttttggggtcgaggtgccgtaaagcactaaatcggaaccctaaagggagcccccgatttagagcttgacggggaaagccggcgaacgtggcgagaaaggaagggaagaaagcgaaaggagcgggcgctagggcgctggcaagtgtagcggtcacgctgcgcgtaaccaccacacccgccgcgcttaatgcgccgctacagggcgcgtcccattcgccattcaggctgcgcaactgttgggaagggcgatcggtgcgggcctcttcgctattacgccagctggcgaaagggggatgtgctgcaaggcgattaagttgggtaacgccagggttttcccagtcacgacgttgttttatcggtctgtatatcgaggtttatttattaatttgaatagatattaagttttattatatttacacttacatactaataataaattcaacaaacaatttatttatgtttatttatttattaaaaaaaaacaaaaactcaaaatttcttctataaagtaacaaaacttttatcgaattcctgcagcccgggggatccactagttctagagggacagcccccccccaaagcccccagggatgtaattacgtccctcccccgctagggggcagcagcgagccgcccggggctccgctccggtccggcgctccccccgcatccccgagccggcagcgtgcggggacagcccgggcacggggaaggtggcacgggatcgctttcctctgaacgcttctcgctgctctttgagcctgcagacacctggggggatacggggaaaaggcctccaaggccagcttcccacaataagttgggtgaattttggctcattcctcctttctataggattgaggtcagagctttgtgatgggaattctgtggaatgtgtgtcagttagggtgtggaaagtcccgacattgattattgactagttattaatagtaatcaattacggggtcattagttcatagcccatatatggagttccgcgttacataacttacggtaaatggcccgcctggctgaccgcccaacgacccccgcccattgacgtcaataatgacgtatgttcccatagtaacgccaatagggactttccattgacgtcaatgggtggagtatttacggtaaactgcccacttggcagtacatcaagtgtatcatatgccaagtacgccccctattgacgtcaatgacggtaaatggcccgcctggcattatgcccagtacatgaccttatgggactttcctacttggcagtacatctacgtattagtcatcgctattaccatggtgatgcggttttggcagtacatcaatgggcgtggatagcggtttgactcacggggatttccaagtctccaccccattgacgtcaatgggagtttgttttggcaccaaaatcaacgggactttccaaaatgtcgtaacaactccgccccattgacgcaaatgggcggtaggcgtgtacggtgggaggtctatataagcagagctggtttagtgaaccgtcagatcagatctttgtcgatcctaccatccactcgacacacccgccagcggccgcagttgcgcagccatcgacgtcagacgcggaagcttcgatcaactacgcagacaggtaccaaaacaaatgttctcgtcacgtgggcatgaatctgatgctgtttccctgcagacaatgcgagagaatgaatcagaattcaaatatctgcttcactcacggacagaaagactgtttagagtgctttcccgtgtcagaatctcaacccgtttctgtcgtcaaaaaggcgtatcagaaactgtgctacattcatcatatcatgggaaaggtgccagacgcttgcactgcctgcgatctggtcaatgtggatttggatgactgcatctttgaacaataaatgatttaaatcaggtatggctgccgatggttatcttccagattggctcgaggacactctctctgaaggaataagacagtggtggaagctcaaacctggcccaccaccaccaaagcccgcagagcggcataaggacgacagcaggggtcttgtgcttcctgggtacaagtacctcggacccttcaacggactcgacaagggagagccggtcaacgaggcagacgccgcggccctcgagcacgacaaagcctacgaccggcagctcgacagcggagacaacccgtacctcaagtacaaccacgccgacgcggagtttcaggagcgccttaaagaagatacgtcttttgggggcaacctcggacgagcagtcttccaggcgaaaaagagggttcttgaacctctgggcctggttgaggaacctgttaagacggctccgggaaaaaagaggccggtagagcactctcctgtggagccagactcctcctcgggaaccggaaaggcgggccagcagcctgcaagaaaaagattgaattttggtcagactggagacgcagactcagtacctgacccccagcctctcggacagccaccagcagccccctctggtctgggaactaatacgatggctacaggcagtggcgcaccaatggcagacaataacgagggcgccgacggagtgggtaattcctcgggaaattggcattgcgattccacatggatgggcgacagagtcatcaccaccagcacccgaacctgggccctgcccacctacaacaaccacctctacaaacaaatttccagccaatcaggagcctcgaacgacaatcactactttggctacagcaccccttgggggtattttgacttcaacagattccactgccacttttcaccacgtgactggcaaagactcatcaacaacaactggggattccgacccaagagactcaacttcaagctctttaacattcaagtcaaagaggtcacgcagaatgacggtacgacgacgattgccaataaccttaccagcacggttcaggtgtttactgactcggagtaccagctcccgtacgtcctcggctcggcgcatcaaggatgcctcccgccgttcccagcagacgtcttcatggtgccacagtatggatacctcaccctgaacaacgggagtcaggcagtaggacgctcttcattttactgcctggagtactttccttctcagatgctgcgtaccggaaacaactttaccttcagctacacttttgaggacgttcctttccacagcagctacgctcacagccagagtctggaccgtctcatgaatcctctcatcgaccagtacctgtattacttgagcagaacaaacactccaagtggaaccaccacgcagtcaaggcttcagttttctcaggccggagcgagtgacattcgggaccagtctaggaactggcttcctggaccctgttaccgccagcagcgagtatcaaagacatctgcggataacaacaacagtgaatactcgtggactggagctaccaagtaccacctcaatggcagagactctctggtgaatccgggcccggccatggcaagccacaaggacgatgaagaaaagttttttcctcagagcggggttctcatctttgggaagcaaggctcagagaaaacaaatgtggacattgaaaaggtcatgattacagacgaagaggaaatcaggacaaccaatcccgtggctacggagcagtatggttctgtatctaccaacctccagagaggcaacagacaagcagctaccgcagatgtcaacacacaaggcgttcttccaggcatggtctggcaggacagagatgtgtaccttcaggggcccatctgggcaaagattccacacacggacggacattttcacccctctcccctcatgggtggattcggacttaaacaccctcctccacagattctcatcaagaacaccccggtacctgcgaatccttcgaccaccttcagtgcggcaaagtttgcttccttcatcacacagtactccacgggacaggtcagcgtggagatcgagtgggagctgcagaaggaaaacagcaaacgctggaatcccgaaattcagtacacttccaactacaacaagtctgttaatgtggactttactgtggacactaatggcgtgtattcagagcctcgccccattggcaccagatacctgactcgtaatctgtaataacccgggagttctagggatctggcggccgctcgagtctagagggcccgtttaaacccgctgatcagcctcgactgtgccttctagttgccagccatctgttgtttgcccctcccccgtgccttccttgaccctggaaggtgccactcccactgtcctttcctaataaaatgaggaaattgcatcgcattgtctgagtaggtgtcattctattctggggggtggggtggggcaggacagcaagggggaggattgggaagacaatagcaggcatgctggggatgcggtgggctctatgggcgatcgctagcgtttaaacttaagcttggtaccgagctcggatccactagtccagtgtggtggaattcctgcttcgcgatgtacgggccagatatacgcgttgtttactcatgtctgggggtgggcgaagaactccagcatgagatccccgcgctggaggatcatccagccggcgtcccggaaaacgattccgaagcccaacctttgcctgcaggtcgactctagaggatccgaaaaaacctcccacacctccccctgaacctgaaacataaaatgaatgcaattgttgttgttaacttgtttattgcagcttataatggttacaaataaagcaatagcatcacaaatttcacaaataaagcatttttttcactgcattctagttgtggtttgtccaaactcatcaatgtatcttatcatgtctggatccccgcggccgcggtacccacgtgggcgcgccatttaaatgataactcagagagagtgtcctcgagccaatctggaagataaccatcggcagccatacctgatttaaatcatttattgttcaaagatgcagtcatccaaatccacattgaccagatcgcaggcagtgcaagcgtctggcacctttcccatgatatgatgaatgtagcacagtttctgatacgcctttttgacgacagaaacgggttgagattctgacacgggaaagcactctaaacagtctttctgtccgtgagtgaagcagatatttgaattctgattcattctctcgcattgtctgcagggaaacagcatcagattcatgcccacgtgacgagaacatttgttttggtacctgtctgcgtagttgatcgaagcttccgcgtctgacgtcgatggctgcgcaactgactcgcgcacccgtttgggctcacttatatctgcgtcactgggggcgggtcttttcttggctccaccctttttgacgtagaattcatgctccacctcaaccacgtgatcctttgcccaccggaaaaagtctttgacttcctgcttggtgaccttcccaaagtcatgatccagacggcgggtgagttcaaatttgaacatccggtcttgcaacggctgctggtgttcgaaggtcgttgagttcccgtcaatcacggcgcacatgttggtgttggaggtgacgatcacgggagtcgggtctatctgggccgaggacttgcatttctggtccacgcgcaccttgcttcctccgagaatggctttggccgactccacgaccttggcggtcatcttcccctcctcccaccagatcaccatcttgtcgacacagtcgttgaagggaaagttctcattggtccagtttacgcacccgtagaagggcacagtgtgggctatggcctccgcgatgttggtcttcccggtagttgcaggcccaaacagccagatggtgttcctcttgccgaactttttcgtggcccatcccagaaagacggaagccgcatattggggatcgtacccgtttagttccaaaattttataaatccgattgctggaaatgtcctccacgggctgctggcccaccaggtagtcgggggcggttttagtcaggctcataatctttcccgcattgtccaaggcagccttgatttgggaccgcgagttggaggccgcattgaaggagatgtatgaggcctggtcctcctggatccactgcttctccgaggtaatccccttgtccacgagccacccgaccagctccatgtacctggctgaagtttttgatctgatcaccggcgcatcagaattgggattctgattctctttgttctgctcctgcgtctgcgacacgtgcgtcagatgctgcgccaccaaccgtttacgctccgtgagattcaaacaggcgcttaaatactgttccatattagtccacgcccactggagctcaggctgggttttggggagcaagtaattggggatgtagcactcatccaccaccttgttcccgcctccggcgccatttctggtctttgtgaccgcgaaccagtttggcaaagtcggctcgatcccgcggtaaattctctgaatcagtttttcgcgaatctgactcaggaaacgtcccaaaaccatggatttcaccccggtggtttccacgagcacgtgcatgtggaagtagctctctcccttctcaaattgcacaaagaaaagggcctccggggccttactcacacggcgccattccgtcagaaagtcgcgctgcagcttctcggccacggtcaggggtgcctgctcaatcagattcagatccatgtcagaatctggcggcaactcccattccttctcggccacccagttcacaaagctgtcagaaatgccgggcagatgctcgtcaaggtcgctggggaccttaatcacaatctcgtaaaaccccggcatggcggcgataactattatcatcgtgtttttcaaaggaaaaccacgtccccgtggttcggggggcctagacgtttttttaacctcgactaaacacatgtaaagcatgtgcaccgaggccccagatcagatcccatacaatggggtaccttctgggcatccttcagccccttgttgaatacgcttgaggagagccatttgactctttccacaactatccaactcacaacgtggcactggggttgtgccgcctttgcaggtgtatcttatacacgtggcttttggccgcagaggcacctgtcgccaggtggggggttccgctgcctgcaaagggtcgctacagacgttgtttgtcttcaagaagcttccagaggaactgcttccttcacgacattcaacagaccttgcattcctttggcgagaggggaaagacccctaggaatgctcgtcaagaagacagggccaggtttccgggccctcacattgccaaaagacggcaatatggtggaaaataacatatagacaaacgcacaccggccttattccaagcggcttcggccagtaacgttagggggggggggcggaattctatccctcagttatctcagagagagtgtcctcgagccaatctggaagataaccatcggcagccatacctgatttaaatcatttattgttcaaagatgcagtcatccaaatccacattgaccagatcgcaggcagtgcaagcgtctggcacctttcccatgatatgatgaatgtagcacagtttctgatacgcctttttgacgacagaaacgggttgagattctgacacgggaaagcactctaaacagtctttctgtccgtgagtgaagcagatatttgaattctgattcattctctcgcattgtctgcagggaaacagcatcagattcatgcccacgtgacgagaacatttgttttggtacctgtctgcgtagttgatcgaagcttccgcgtctgacgtcgatggctgcgcaactgactcgcgcacccgtttgggctcacttatatctgcgtcactgggggcgggtcttttcttggctccaccctttttgacgtagaattcatgctccacctcaaccacgtgatcctttgcccaccggaaaaagtctttgacttcctgcttggtgaccttcccaaagtcatgatccagacggcgggtgagttcaaatttgaacatccggtcttgcaacggctgctggtgttcgaaggtcgttgagttcccgtcaatcacggcgcacatgttggtgttggaggtgacgatcacgggagtcgggtctatctgggccgaggacttgcatttctggtccacgcgcaccttgcttcctccgagaatggctttggccgactccacgaccttggcggtcatcttcccctcctcccaccagatcaccatcttgtcgacacagtcgttgaagggaaagttctcattggtccagtttacgcacccgtagaagggcacagtgtgggctatggcctccgcgatgttggtcttcccggtagttgcaggcccaaacagccagatggtgttcctcttgccgaactttttcgtggcccatcccagaaagacggaagccgcatattggggatcgtacccgtttagttccaaaattttataaatccgattgctggaaatgtcctccacgggctgctggcccaccaggtagtcgggggcggttttagtcaggctcataatctttcccgcattgtccaaggcagccttgatttgggaccgcgagttggaggccgcattgaaggagatgtatgaggcctggtcctcctggatccactgcttctccgaggtaatccccttgtccacgagccacccgaccagctccatggtggcttcggggccgcggaggctggatcggtcccggtgtcttctatggaggtcaaaacagcgtggatggcgtctccaggcgatctgacggttcactaaacgagctctgcttatatagacctcccaccgtacacgcctaccgcccatttgcgtcaatggggcggagttgttacgacattttggaaagtcccgttgattttggtgccaaaacaaactcccattgacgtcaatggggtggagacttggaaatccccgtgagtcaaaccgctatccacgcccattgatgtactgccaaaaccgcatcaccatggtaatagcgatgactaatacgtagatgtactgccaagtaggaaagtcccataaggtcatgtactgggcataatgccaggcgggccatttaccgtcattgacgtcaatagggggcgtacttggcatatgatacacttgatgtactgccaagtgggcagtttaccgtaaatactccacccattgacgtcaatggaaagtccctattggcgttactatgggaacatacgtcattattgacgtcaatgggcgggggtcgttgggcggtcagccaggcgggccatttaccgtaagttatgtaacgcggaactccatatatgggctatgaactaatgaccccgtaattgattactattaataactagtcaataatcaatgtcttacatccctgggggctttgggggggggctgtccctctagagcggccgccaccgcggtggagctccagcttttgttccctttagtgagggttaattagatcttaatacgactcactatagggcgaattgggtaccgggccccccctcgaggtcgacggtatcgtgtgaaattgttatccgctcacaattccacacaacatacgagccggaagcataaagtgtaaagcctggggtgcctaatgagtgagctaactcacattaattgcgttgcgctcactgcccgctttccagtcgggaaacctgtcgtgccagctgcattaatgaatcggccaacgcgcggggagaggcggtttgcgtattgggcgctcttccgcttcctcgctcactgactcgctgcgctcggtcgttcggctgcggcgagcggtatcagctcactcaaaggcggtaatacggttatccacagaatcaggggataacgcaggaaagaacatgtgagcaaaaggccagcaaaaggccaggaaccgtaaaaaggccgcgttgctggcgtt

SEQ ID NO: 3 - DNA, 11920 bp, synthetic construct
  misc_feature 1..11920: note = plasmid
  source 1..11920: mol_type = other DNA
atgactctcttaaggtagccaaatttccataggctccgcccccctgacgagcatcacaaaaatcgacgctcaagtcagaggtggcgaaacccgacaggactataaagataccaggcgtttccccctggaagctccctcgtgcgctctcctgttccgaccctgccgcttaccggatacctgtccgcctttctcccttcgggaagcgtggcgctttctcatagctcacgctgtaggtatctcagttcggtgtaggtcgttcgctccaagctgggctgtgtgcacgaaccccccgttcagcccgaccgctgcgccttatccggtaactatcgtcttgagtccaacccggtaagacacgacttatcgccactggcagcagccactggtaacaggattagcagagcgaggtatgtaggcggtgctacagagttcttgaagtggtggcctaactacggctacactagaaggacagtatttggtatctgcgctctgctgaagccagttaccttcggaaaaagagttggtagctcttgatccggcaaacaaaccaccgctggtagcggtggtttttttgtttgcaagcagcagattacgcgcagaaaaaaaggatctcaagaagatcctttgatcttttctacggggtctgacgctcagtggaacgaaaactcacgttaagggattttggtcatgagattatcaaaaaggatcttcacctagatccttttaaattaaaaatgaagttttaaatcaatctaaagtatatatgagtaaacttggtctgacagttaccaatgcttaatcagtgaggcacctatctcagcgatctgtctatttcgttcatccatagttgcctgactccccgtcgtgtagataactacgatacgggagggcttaccatctggccccagtgctgcaatgataccgcgagacccacgctcaccggctccagatttatcagcaataaaccagccagccggaagggccgagcgcagaagtggtcctgcaactttatccgcctccatccagtctattaattgttgccgggaagctagagtaagtagttcgccagttaatagtttgcgcaacgttgttgccattgctacaggcatcgtggtgtcacgctcgtcgtttggtatggcttcattcagctccggttcccaacgatcaaggcgagttacatgatcccccatgttgtgcaaaaaagcggttagctccttcggtcctccgatcgttgtcagaagtaagttggccgcagtgttatcactcatggttatggcagcactgcataattctcttactgtcatgccatccgtaagatgcttttctgtgactggtgagtactcaaccaagtcattctgagaatagtgtatgcggcgaccgagttgctcttgcccggcgtcaatacgggataataccgcgccacatagcagaactttaaaagtgctcatcattggaaaacgttcttcggggcgaaaactctcaaggatcttaccgctgttgagatccagttcgatgtaacccactcgtgcacccaactgatcttcagcatcttttactttcaccagcgtttctgggtgagcaaaaacaggaaggcaaaatgccgcaaaaaagggaataagggcgacacggaaatgttgaatactcatactcttcctttttcaatattattgaagcatttatcagggttattgtctcatgagcggatacatatttgaatgtatttagaaaaataaacaaataggggttccgcgcacatttccccgaaaagtgccacctaaattgtaagcgttaatattttgttaaaattcgcgttaaatttttgttaaatcagctcattttttaaccaataggccgaaatcggcaaaatcccttataaatcaaaagaatagaccgagatagggttgagtgttgttccagtttggaacaagagtccactattaaagaacgtggactccaacgtcaaagggcgaaaaaccgtctatcagggcgatggcccactacgtgaaccatcaccctaatcaagttttttggggtcgaggtgccgtaaagcactaaatcggaaccctaaagggagcccccgatttagagcttgacggggaaagccggcgaacgtggcgagaaaggaagggaagaaagcgaaaggagcgggcgctagggcgctggcaagtgtagcggtcacgctgcgcgtaaccaccacacccgccgcgcttaatgcgccgctacagggcgcgtcccattcgccattcaggctgcgcaactgttgggaagggcgatcggtgcgggcctcttcgctattacgccagctggcgaaagggggatgtgctgcaaggcgattaagttgggtaacgccagggttttcccagtcacgacgttgttttatcggtctgtatatcgaggtttatttattaatttgaatagatattaagttttattatatttacacttacatactaataataaattcaacaaacaatttatttatgtttatttatttattaaaaaaaaacaaaaactcaaaatttcttctataaagtaacaaaacttttatcgaattcctgcagcccgggggatccactagttctagagggacagcccccccccaaagcccccagggatgtaattacgtccctcccccgctagggggcagcagcgagccgcccggggctccgctccggtccggcgctccccccgcatccccgagccggcagcgtgcggggacagcccgggcacggggaaggtggcacgggatcgctttcctctgaacgcttctcgctgctctttgagcctgcagacacctggggggatacggggaaaaggcctccaaggccagcttcccacaataagttgggtgaattttggctcattcctcctttctataggattgaggtcagagctttgtgatgggaattctgtggaatgtgtgtcagttagggtgtggaaagtcccgacattgattattgactagttattaatagtaatcaattacggggtcattagttcatagcccatatatggagttccgcgttacataacttacggtaaatggcccgcctggctgaccgcccaacgacccccgcccattgacgtcaataatgacgtatgttcccatagtaacgccaatagggactttccattgacgtcaatgggtggagtatttacggtaaactgcccacttggcagtacatcaagtgtatcatatgccaagtacgccccctattgacgtcaatgacggtaaatggcccgcctggcattatgcccagtacatgaccttatgggactttcctacttggcagtacatctacgtattagtcatcgctattaccatggtgatgcggttttggcagtacatcaatgggcgtggatagcggtttgactcacggggatttccaagtctccaccccattgacgtcaatgggagtttgttttggcaccaaaatcaacgggactttccaaaatgtcgtaacaactccgccccattgacgcaaatgggcggtaggcgtgtacggtgggaggtctatataagcagagctggtttagtgaaccgtcagatcagatctttgtcgatcctaccatccactcgacacacccgccagcggccgcagttgcgcagccatcgacgtcagacgcggaagcttcgatcaactacgcagacaggtaccaaaacaaatgttctcgtcacgtgggcatgaatctgatgctgtttccctgcagacaatgcgagagaatgaatcagaattcaaatatctgcttcactcacggacagaaagactgtttagagtgctttcccgtgtcagaatctcaacccgtttctgtcgtcaaaaaggcgtatcagaaactgtgctacattcatcatatcatgggaaaggtgccagacgcttgcactgcctgcgatctggtcaatgtggatttggatgactgcatctttgaacaataaatgatttaaatcaggtatgtcttttgttgatcaccctccagattggttggaagaagttggtgaaggtcttcgcgagtttttgggccttgaagcgggcccaccgaaaccaaaacccaatcagcagcatcaagatcaagcccgtggtcttgtgctgcctggttataactatctcggacccggaaacggtctcgatcgaggagagcctgtcaacagggcagacgaggtcgcgcgagagcacgacatctcgtacaacgagcagcttgaggcgggagacaacccctacctcaagtacaaccacgcggacgccgagtttcaggagaagctcgccgacgacacatccttcgggggaaacctcggaaaggcagtctttcaggccaagaaaagggttctcgaaccttttggcctggttgaagagggtgctaagacggcccctaccggaaagcggatagacgaccactttccaaaaagaaagaaggctcggaccgaagaggactccaagccttccacctcgtcagacgccgaagctggacccagcggatcccagcagctgcaaatcccagcccaaccagcctcaagtttgggagctgatacaatgtctgcgggaggtggcggcccattgggcgacaataaccaaggtgccgatggagtgggcaatgcctcgggagattggcattgcgattccacgtggatgggggacagagtcgtcaccaagtccacccgaacctgggtgctgcccagctacaacaaccaccagtaccgagagatcaaaagcggctccgtcgacggaagcaacgccaacgcctactttggatacagcaccccctgggggtactttgactttaaccgcttccacagccactggagcccccgagactggcaaagactcatcaacaactactggggcttcagaccccggtccctcagagtcaaaatcttcaacattcaagtcaaagaggtcacggtgcaggactccaccaccaccatcgccaacaacctcacctccaccgtccaagtgtttacggacgacgactaccagctgccctacgtcgtcggcaacgggaccgagggatgcctgccggccttccctccgcaggtctttacgctgccgcagtacggttacgcgacgctgaaccgcgacaacacagaaaatcccaccgagaggagcagcttcttctgcctagagtactttcccagcaagatgctgagaacgggcaacaactttgagtttacctacaactttgaggaggtgcccttccactccagcttcgctcccagtcagaacctgttcaagctggccaacccgctggtggaccagtacttgtaccgcttcgtgagcacaaataacactggcggagtccagttcaacaagaacctggccgggagatacgccaacacctacaaaaactggttcccggggcccatgggccgaacccagggctggaacctgggctccggggtcaaccgcgccagtgtcagcgccttcgccacgaccaataggatggagctcgagggcgcgagttaccaggtgcccccgcagccgaacggcatgaccaacaacctccagggcagcaacacctatgccctggagaacactatgatcttcaacagccagccggcgaacccgggcaccaccgccacgtacctcgagggcaacatgctcatcaccagcgagagcgagacgcagccggtgaaccgcgtggcgtacaacgtcggcgggcagatggccaccaacaaccagagctccaccactgcccccgcgaccggcacgtacaacctccaggaaatcgtgcccggcagcgtgtggatggagagggacgtgtacctccaaggacccatctgggccaagatcccagagacgggggcgcactttcacccctctccggccatgggcggattcggactcaaacacccaccgcccatgatgctcatcaagaacacgcctgtgcccggaaatatcaccagcttctcggacgtgcccgtcagcagcttcatcacccagtacagcaccgggcaggtcaccgtggagatggagtgggagctcaagaaggaaaactccaagaggtggaacccagagatccagtacacaaacaactacaacgacccccagtttgtggactttgccccggacagcaccggggaatacagaaccaccagacctatcggaacccgataccttacccgacccctttaacccgggagttctagggatctggcggccgctcgagtctagagggcccgtttaaacccgctgatcagcctcgactgtgccttctagttgccagccatctgttgtttgcccctcccccgtgccttccttgaccctggaaggtgccactcccactgtcctttcctaataaaatgaggaaattgcatcgcattgtctgagtaggtgtcattctattctggggggtggggtggggcaggacagcaagggggaggattgggaagacaatagcaggcatgctggggatgcggtgggctctatgggcgatcgctagcgtttaaacttaagcttggtaccgagctcggatccactagtccagtgtggtggaattcctgcttcgcgatgtacgggccagatatacgcgttgtttactcatgtctgggggtgggcgaagaactccagcatgagatccccgcgctggaggatcatccagccggcgtcccggaaaacgattccgaagcccaacctttgcctgcaggtcgactctagaggatccgaaaaaacctcccacacctccccctgaacctgaaacataaaatgaatgcaattgttgttgttaacttgtttattgcagcttataatggttacaaataaagcaatagcatcacaaatttcacaaataaagcatttttttcactgcattctagttgtggtttgtccaaactcatcaatgtatcttatcatgtctggatccccgcggccgcggtacccacgtgggcgcgccatttaaatgataactcagagagagtgtcctcgagccaatctggaagataaccatcggcagccatacctgatttaaatcatttattgttcaaagatgcagtcatccaaatccacattgaccagatcgcaggcagtgcaagcgtctggcacctttcccatgatatgatgaatgtagcacagtttctgatacgcctttttgacgacagaaacgggttgagattctgacacgggaaagcactctaaacagtctttctgtccgtgagtgaagcagatatttgaattctgattcattctctcgcattgtctgcagggaaacagcatcagattcatgcccacgtgacgagaacatttgttttggtacctgtctgcgtagttgatcgaagcttccgcgtctgacgtcgatggctgcgcaactgactcgcgcacccgtttgggctcacttatatctgcgtcactgggggcgggtcttttcttggctccaccctttttgacgtagaattcatgctccacctcaaccacgtgatcctttgcccaccggaaaaagtctttgacttcctgcttggtgaccttcccaaagtcatgatccagacggcgggtgagttcaaatttgaacatccggtcttgcaacggctgctggtgttcgaaggtcgttgagttcccgtcaatcacggcgcacatgttggtgttggaggtgacgatcacgggagtcgggtctatctgggccgaggacttgcatttctggtccacgcgcaccttgcttcctccgagaatggctttggccgactccacgaccttggcggtcatcttcccctcctcccaccagatcaccatcttgtcgacacagtcgttgaagggaaagttctcattggtccagtttacgcacccgtagaagggcacagtgtgggctatggcctccgcgatgttggtcttcccggtagttgcaggcccaaacagccagatggtgttcctcttgccgaactttttcgtggcccatcccagaaagacggaagccgcatattggggatcgtacccgtttagttccaaaattttataaatccgattgctggaaatgtcctccacgggctgctggcccaccaggtagtcgggggcggttttagtcaggctcataatctttcccgcattgtccaaggcagccttgatttgggaccgcgagttggaggccgcattgaaggagatgtatgaggcctggtcctcctggatccactgcttctccgaggtaatccccttgtccacgagccacccgaccagctccatgtacctggctgaagtttttgatctgatcaccggcgcatcagaattgggattctgattctctttgttctgctcctgcgtctgcgacacgtgcgtcagatgctgcgccaccaaccgtttacgctccgtgagattcaaacaggcgcttaaatactgttccatattagtccacgcccactggagctcaggctgggttttggggagcaagtaattggggatgtagcactcatccaccaccttgttcccgcctccggcgccatttctggtctttgtgaccgcgaaccagtttggcaaagtcggctcgatcccgcggtaaattctctgaatcagtttttcgcgaatctgactcaggaaacgtcccaaaaccatggatttcaccccggtggtttccacgagcacgtgcatgtggaagtagctctctcccttctcaaattgcacaaagaaaagggcctccggggccttactcacacggcgccattccgtcagaaagtcgcgctgcagcttctcggccacggtcaggggtgcctgctcaatcagattcagatccatgtcagaatctggcggcaactcccattccttctcggccacccagttcacaaagctgtcagaaatgccgggcagatgctcgtcaaggtcgctggggaccttaatcacaatctcgtaaaaccccggcatggcggcgataactattatcatcgtgtttttcaaaggaaaaccacgtccccgtggttcggggggcctagacgtttttttaacctcgactaaacacatgtaaagcatgtgcaccgaggccccagatcagatcccatacaatggggtaccttctgggcatccttcagccccttgttgaatacgcttgaggagagccatttgactctttccacaactatccaactcacaacgtggcactggggttgtgccgcctttgcaggtgtatcttatacacgtggcttttggccgcagaggcacctgtcgccaggtggggggttccgctgcctgcaaagggtcgctacagacgttgtttgtcttcaagaagcttccagaggaactgcttccttcacgacattcaacagaccttgcattcctttggcgagaggggaaagacccctaggaatgctcgtcaagaagacagggccaggtttccgggccctcacattgccaaaagacggcaatatggtggaaaataacatatagacaaacgcacaccggccttattccaagcggcttcggccagtaacgttagggggggggggcggaattctatccctcagttatctcagagagagtgtcctcgagccaatctggaagataaccatcggcagccatacctgatttaaatcatttattgttcaaagatgcagtcatccaaatccacattgaccagatcgcaggcagtgcaagcgtctggcacctttcccatgatatgatgaatgtagcacagtttctgatacgcctttttgacgacagaaacgggttgagattctgacacgggaaagcactctaaacagtctttctgtccgtgagtgaagcagatatttgaattctgattcattctctcgcattgtctgcagggaaacagcatcagattcatgcccacgtgacgagaacatttgttttggtacctgtctgcgtagttgatcgaagcttccgcgtctgacgtcgatggctgcgcaactgactcgcgcacccgtttgggctcacttatatctgcgtcactgggggcgggtcttttcttggctccaccctttttgacgtagaattcatgctccacctcaaccacgtgatcctttgcccaccggaaaaagtctttgacttcctgcttggtgaccttcccaaagtcatgatccagacggcgggtgagttcaaatttgaacatccggtcttgcaacggctgctggtgttcgaaggtcgttgagttcccgtcaatcacggcgcacatgttggtgttggaggtgacgatcacgggagtcgggtctatctgggccgaggacttgcatttctggtccacgcgcaccttgcttcctccgagaatggctttggccgactccacgaccttggcggtcatcttcccctcctcccaccagatcaccatcttgtcgacacagtcgttgaagggaaagttctcattggtccagtttacgcacccgtagaagggcacagtgtgggctatggcctccgcgatgttggtcttcccggtagttgcaggcccaaacagccagatggtgttcctcttgccgaactttttcgtggcccatcccagaaagacggaagccgcatattggggatcgtacccgtttagttccaaaattttataaatccgattgctggaaatgtcctccacgggctgctggcccaccaggtagtcgggggcggttttagtcaggctcataatctttcccgcattgtccaaggcagccttgatttgggaccgcgagttggaggccgcattgaaggagatgtatgaggcctggtcctcctggatccactgcttctccgaggtaatccccttgtccacgagccacccgaccagctccatggtggcttcggggccgcggaggctggatcggtcccggtgtcttctatggaggtcaaaacagcgtggatggcgtctccaggcgatctgacggttcactaaacgagctctgcttatatagacctcccaccgtacacgcctaccgcccatttgcgtcaatggggcggagttgttacgacattttggaaagtcccgttgattttggtgccaaaacaaactcccattgacgtcaatggggtggagacttggaaatccccgtgagtcaaaccgctatccacgcccattgatgtactgccaaaaccgcatcaccatggtaatagcgatgactaatacgtagatgtactgccaagtaggaaagtcccataaggtcatgtactgggcataatgccaggcgggccatttaccgtcattgacgtcaatagggggcgtacttggcatatgatacacttgatgtactgccaagtgggcagtttaccgtaaatactccacccattgacgtcaatggaaagtccctattggcgttactatgggaacatacgtcattattgacgtcaatgggcgggggtcgttgggcggtcagccaggcgggccatttaccgtaagttatgtaacgcggaactccatatatgggctatgaactaatgaccccgtaattgattactattaataactagtcaataatcaatgtcttacatccctgggggctttgggggggggctgtccctctagagcggccgccaccgcggtggagctccagcttttgttccctttagtgagggttaattagatcttaatacgactcactatagggcgaattgggtaccgggccccccctcgaggtcgacggtatcgtgtgaaattgttatccgctcacaattccacacaacatacgagccggaagcataaagtgtaaagcctggggtgcctaatgagtgagctaactcacattaattgcgttgcgctcactgcccgctttccagtcgggaaacctgtcgtgccagctgcattaatgaatcggccaacgcgcggggagaggcggtttgcgtattgggcgctcttccgcttcctcgctcactgactcgctgcgctcggtcgttcggctgcggcgagcggtatcagctcactcaaaggcggtaatacggttatccacagaatcaggggataacgcaggaaagaacatgtgagcaaaaggccagcaaaaggccaggaaccgtaaaaaggccgcgttgctggcgtt

SEQ ID NO: 4 - DNA, 11959 bp, synthetic construct
  misc_feature 1..11959: note = plasmid
  source 1..11959: mol_type = other DNA
atgactctcttaaggtagccaaatttccataggctccgcccccctgacgagcatcacaaaaatcgacgctcaagtcagaggtggcgaaacccgacaggactataaagataccaggcgtttccccctggaagctccctcgtgcgctctcctgttccgaccctgccgcttaccggatacctgtccgcctttctcccttcgggaagcgtggcgctttctcatagctcacgctgtaggtatctcagttcggtgtaggtcgttcgctccaagctgggctgtgtgcacgaaccccccgttcagcccgaccgctgcgccttatccggtaactatcgtcttgagtccaacccggtaagacacgacttatcgccactggcagcagccactggtaacaggattagcagagcgaggtatgtaggcggtgctacagagttcttgaagtggtggcctaactacggctacactagaaggacagtatttggtatctgcgctctgctgaagccagttaccttcggaaaaagagttggtagctcttgatccggcaaacaaaccaccgctggtagcggtggtttttttgtttgcaagcagcagattacgcgcagaaaaaaaggatctcaagaagatcctttgatcttttctacggggtctgacgctcagtggaacgaaaactcacgttaagggattttggtcatgagattatcaaaaaggatcttcacctagatccttttaaattaaaaatgaagttttaaatcaatctaaagtatatatgagtaaacttggtctgacagttaccaatgcttaatcagtgaggcacctatctcagcgatctgtctatttcgttcatccatagttgcctgactccccgtcgtgtagataactacgatacgggagggcttaccatctggccccagtgctgcaatgataccgcgagacccacgctcaccggctccagatttatcagcaataaaccagccagccggaagggccgagcgcagaagtggtcctgcaactttatccgcctccatccagtctattaattgttgccgggaagctagagtaagtagttcgccagttaatagtttgcgcaacgttgttgccattgctacaggcatcgtggtgtcacgctcgtcgtttggtatggcttcattcagctccggttcccaacgatcaaggcgagttacatgatcccccatgttgtgcaaaaaagcggttagctccttcggtcctccgatcgttgtcagaagtaagttggccgcagtgttatcactcatggttatggcagcactgcataattctcttactgtcatgccatccgtaagatgcttttctgtgactggtgagtactcaaccaagtcattctgagaatagtgtatgcggcgaccgagttgctcttgcccggcgtcaatacgggataataccgcgccacatagcagaactttaaaagtgctcatcattggaaaacgttcttcggggcgaaaactctcaaggatcttaccgctgttgagatccagttcgatgtaacccactcgtgcacccaactgatcttcagcatcttttactttcaccagcgtttctgggtgagcaaaaacaggaaggcaaaatgccgcaaaaaagggaataagggcgacacggaaatgttgaatactcatactcttcctttttcaatattattgaagcatttatcagggttattgtctcatgagcggatacatatttgaatgtatttagaaaaataaacaaataggggttccgcgcacatttccccgaaaagtgccacctaaattgtaagcgttaatattttgttaaaattcgcgttaaatttttgttaaatcagctcattttttaaccaataggccgaaatcggcaaaatcccttataaatcaaaagaatagaccgagatagggttgagtgttgttccagtttggaacaagagtccactattaaagaacgtggactccaacgtcaaagggcgaaaaaccgtctatcagggcgatggcccactacgtgaaccatcaccctaatcaagttttttggggtcgaggtgccgtaaagcactaaatcggaaccctaaagggagcccccgatttagagcttgacggggaaagccggcgaacgtggcgagaaaggaagggaagaaagcgaaaggagcgggcgctagggcgctggcaagtgtagcggtcacgctgcgcgtaaccaccacacccgccgcgcttaatgcgccgctacagggcgcgtcccattcgccattcaggctgcgcaactgttgggaagggcgatcggtgcgggcctcttcgctattacgccagctggcgaaagggggatgtgctgcaaggcgattaagttgggtaacgccagggttttcccagtcacgacgttgttttatcggtctgtatatcgaggtttatttattaatttgaatagatattaagttttattatatttacacttacatactaataataaattcaacaaacaatttatttatgtttatttatttattaaaaaaaaacaaaaactcaaaatttcttctataaagtaacaaaacttttatcgaattcctgcagcccgggggatccactagttctagagggacagcccccccccaaagcccccagggatgtaattacgtccctcccccgctagggggcagcagcgagccgcccggggctccgctccggtccggcgctccccccgcatccccgagccggcagcgtgcggggacagcccgggcacggggaaggtggcacgggatcgctttcctctgaacgcttctcgctgctctttgagcctgcagacacctggggggatacggggaaaaggcctccaaggccagcttcccacaataagttgggtgaattttggctcattcctcctttctataggattgaggtcagagctttgtgatgggaattctgtggaatgtgtgtcagttagggtgtggaaagtcccgacattgattattgactagttattaatagtaatcaattacggggtcattagttcatagcccatatatggagttccgcgttacataacttacggtaaatggcccgcctggctgaccgcccaacgacccccgcccattgacgtcaataatgacgtatgttcccatagtaacgccaatagggactttccattgacgtcaatgggtggagtatttacggtaaactgcccacttggcagtacatcaagtgtatcatatgccaagtacgccccctattgacgtcaatgacggtaaatggcccgcctggcattatgcccagtacatgaccttatgggactttcctacttggcagtacatctacgtattagtcatcgctattaccatggtgatgcggttttggcagtacatcaatgggcgtggatagcggtttgactcacggggatttccaagtctccaccccattgacgtcaatgggagtttgttttggcaccaaaatcaacgggactttccaaaatgtcgtaacaactccgccccattgacgcaaatgggcggtaggcgtgtacggtgggaggtctatataagcagagctggtttagtgaaccgtcagatcagatctttgtcgatcctaccatccactcgacacacccgccagcggccgcagttgcgcagccatcgacgtcagacgcggaagcttcgatcaactacgcagacaggtaccaaaacaaatgttctcgtcacgtgggcatgaatctgatgctgtttccctgcagacaatgcgagagaatgaatcagaattcaaatatctgcttcactcacggacagaaagactgtttagagtgctttcccgtgtcagaatctcaacccgtttctgtcgtcaaaaaggcgtatcagaaactgtgctacattcatcatatcatgggaaaggtgccagacgcttgcactgcctgcgatctggtcaatgtggatttggatgactgcatctttgaacaataaatgatttaaatcaggtatggctgccgatggttatcttccagattggctcgaggacaacctctctgagggcattcgcgagtggtgggacttgaaacctggagccccgaaacccaaagccaaccagcaaaagcaggacgacggccggggtctggtgcttcctggctacaagtacctcggacccttcaacggactcgacaagggggagcccgtcaacgcggcggatgcagcggccctcgagcacgacaaggcctacgaccagcagctcaaagcgggtgacaatccgtacctgcggtataaccacgccgacgccgagtttcaggagcgtctgcaagaagatacgtcttttgggggcaacctcgggcgagcagtcttccaggccaagaagagggttctcgaaccttttggtctggttgaggaaggtgctaagacggctcctggaaagaaacgtccggtagagcagtcgccacaagagccagactcctcctcgggcattggcaagacaggccagcagcccgctaaaaagagactcaattttggtcagactggcgactcagagtcagtccccgacccacaacctctcggagaacctccagcaacccccgctgctgtgggacctactacaatggcttcaggcggtggcgcaccaatggcagacaataacgaaggcgccgacggagtgggtaatgcctcaggaaattggcattgcgattccacatggctgggcgacagagtcatcaccaccagcacccgaacatgggccttgcccacctataacaaccacctctacaagcaaatctccagtgcttcaacgggggccagcaacgacaaccactacttcggctacagcaccccctgggggtattttgatttcaacagattccactgccatttctcaccacgtgactggcagcgactcatcaacaacaattggggattccggcccaagagactcaacttcaagctcttcaacatccaagtcaaggaggtcacgacgaatgatggcgtcacgaccatcgctaataaccttaccagcacggttcaagtcttctcggactcggagtaccagttgccgtacgtcctcggctctgcgcaccagggctgcctccctccgttcccggcggacgtgttcatgattccgcagtacggctacctaacgctcaacaatggcagccaggcagtgggacggtcatccttttactgcctggaatatttcccatcgcagatgctgagaacgggcaataactttaccttcagctacaccttcgaggacgtgcctttccacagcagctacgcgcacagccagagcctggaccggctgatgaatcctctcatcgaccagtacctgtattacctgaacagaactcagaatcagtccggaagtgcccaaaacaaggacttgctgtttagccgggggtctccagctggcatgtctgttcagcccaaaaactggctacctggaccctgttaccggcagcagcgcgtttctaaaacaaaaacagacaacaacaacagcaactttacctggactggtgcttcaaaatataaccttaatgggcgtgaatctataatcaaccctggcactgctatggcctcacacaaagacgacaaagacaagttctttcccatgagcggtgtcatgatttttggaaaggagagcgccggagcttcaaacactgcattggacaatgtcatgatcacagacgaagaggaaatcaaagccactaaccccgtggccaccgaaagatttgggactgtggcagtcaatctccagagcagcagcacagaccctgcgaccggagatgtgcatgttatgggagccttacctggaatggtgtggcaagacagagacgtatacctgcagggtcctatttgggccaaaattcctcacacggatggacactttcacccgtctcctctcatgggcggctttggacttaagcacccgcctcctcagatcctcatcaaaaacacgcctgttcctgcgaatcctccggcagagttttcggctacaaagtttgcttcattcatcacccagtattccacaggacaagtgagcgtggagattgaatgggagctgcagaaagaaaacagcaaacgctggaatcccgaagtgcagtatacatctaactatgcaaaatctgccaacgttgatttcactgtggacaacaatggactttatactgagcctcgccccattggcacccgttacctcacccgtcccctgtaataacccgggagttctagggatctggcggccgctcgagtctagagggcccgtttaaacccgctgatcagcctcgactgtgccttctagttgccagccatctgttgtttgcccctcccccgtgccttccttgaccctggaaggtgccactcccactgtcctttcctaataaaatgaggaaattgcatcgcattgtctgagtaggtgtcattctattctggggggtggggtggggcaggacagcaagggggaggattgggaagacaatagcaggcatgctggggatgcggtgggctctatgggcgatcgctagcgtttaaacttaagcttggtaccgagctcggatccactagtccagtgtggtggaattcctgcttcgcgatgtacgggccagatatacgcgttgtttactcatgtctgggggtgggcgaagaactccagcatgagatccccgcgctggaggatcatccagccggcgtcccggaaaacgattccgaagcccaacctttgcctgcaggtcgactctagaggatccgaaaaaacctcccacacctccccctgaacctgaaacataaaatgaatgcaattgttgttgttaacttgtttattgcagcttataatggttacaaataaagcaatagcatcacaaatttcacaaataaagcatttttttcactgcattctagttgtggtttgtccaaactcatcaatgtatcttatcatgtctggatccccgcggccgcggtacccacgtgggcgcgccatttaaatgataactcagagagagtgtcctcgagccaatctggaagataaccatcggcagccatacctgatttaaatcatttattgttcaaagatgcagtcatccaaatccacattgaccagatcgcaggcagtgcaagcgtctggcacctttcccatgatatgatgaatgtagcacagtttctgatacgcctttttgacgacagaaacgggttgagattctgacacgggaaagcactctaaacagtctttctgtccgtgagtgaagcagatatttgaattctgattcattctctcgcattgtctgcagggaaacagcatcagattcatgcccacgtgacgagaacatttgttttggtacctgtctgcgtagttgatcgaagcttccgcgtctgacgtcgatggctgcgcaactgactcgcgcacccgtttgggctcacttatatctgcgtcactgggggcgggtcttttcttggctccaccctttttgacgtagaattcatgctccacctcaaccacgtgatcctttgcccaccggaaaaagtctttgacttcctgcttggtgaccttcccaaagtcatgatccagacggcgggtgagttcaaatttgaacatccggtcttgcaacggctgctggtgttcgaaggtcgttgagttcccgtcaatcacggcgcacatgttggtgttggaggtgacgatcacgggagtcgggtctatctgggccgaggacttgcatttctggtccacgcgcaccttgcttcctccgagaatggctttggccgactccacgaccttggcggtcatcttcccctcctcccaccagatcaccatcttgtcgacacagtcgttgaagggaaagttctcattggtccagtttacgcacccgtagaagggcacagtgtgggctatggcctccgcgatgttggtcttcccggtagttgcaggcccaaacagccagatggtgttcctcttgccgaactttttcgtggcccatcccagaaagacggaagccgcatattggggatcgtacccgtttagttccaaaattttataaatccgattgctggaaatgtcctccacgggctgctggcccaccaggtagtcgggggcggttttagtcaggctcataatctttcccgcattgtccaaggcagccttgatttgggaccgcgagttggaggccgcattgaaggagatgtatgaggcctggtcctcctggatccactgcttctccgaggtaatccccttgtccacgagccacccgaccagctccatgtacctggctgaagtttttgatctgatcaccggcgcatcagaattgggattctgattctctttgttctgctcctgcgtctgcgacacgtgcgtcagatgctgcgccaccaaccgtttacgctccgtgagattcaaacaggcgcttaaatactgttccatattagtccacgcccactggagctcaggctgggttttggggagcaagtaattggggatgtagcactcatccaccaccttgttcccgcctccggcgccatttctggtctttgtgaccgcgaaccagtttggcaaagtcggctcgatcccgcggtaaattctctgaatcagtttttcgcgaatctgactcaggaaacgtcccaaaaccatggatttcaccccggtggtttccacgagcacgtgcatgtggaagtagctctctcccttctcaaattgcacaaagaaaagggcctccggggccttactcacacggcgccattccgtcagaaagtcgcgctgcagcttctcggccacggtcaggggtgcctgctcaatcagattcagatccatgtcagaatctggcggcaactcccattccttctcggccacccagttcacaaagctgtcagaaatgccgggcagatgctcgtcaaggtcgctggggaccttaatcacaatctcgtaaaaccccggcatggcggcgataactattatcatcgtgtttttcaaaggaaaaccacgtccccgtggttcggggggcctagacgtttttttaacctcgactaaacacatgtaaagcatgtgcaccgaggccccagatcagatcccatacaatggggtaccttctgggcatccttcagccccttgttgaatacgcttgaggagagccatttgactctttccacaactatccaactcacaacgtggcactggggttgtgccgcctttgcaggtgtatcttatacacgtggcttttggccgcagaggcacctgtcgccaggtggggggttccgctgcctgcaaagggtcgctacagacgttgtttgtcttcaagaagcttccagaggaactgcttccttcacgacattcaacagaccttgcattcctttggcgagaggggaaagacccctaggaatgctcgtcaagaagacagggccaggtttccgggccctcacattgccaaaagacggcaatatggtggaaaataacatatagacaaacgcacaccggccttattccaagcggcttcggccagtaacgttagggggggggggcggaattctatccctcagttatctcagagagagtgtcctcgagccaatctggaagataaccatcggcagccatacctgatttaaatcatttattgttcaaagatgcagtcatccaaatccacattgaccagatcgcaggcagtgcaagcgtctggcacctttcccatgatatgatgaatgtagcacagtttctgatacgcctttttgacgacagaaacgggttgagattctgacacgggaaagcactctaaacagtctttctgtccgtgagtgaagcagatatttgaattctgattcattctctcgcattgtctgcagggaaacagcatcagattcatgcccacgtgacgagaacatttgttttggtacctgtctgcgtagttgatcgaagcttccgcgtctgacgtcgatggctgcgcaactgactcgcgcacccgtttgggctcacttatatctgcgtcactgggggcgggtcttttcttggctccaccctttttgacgtagaattcatgctccacctcaaccacgtgatcctttgcccaccggaaaaagtctttgacttcctgcttggtgaccttcccaaagtcatgatccagacggcgggtgagttcaaatttgaacatccggtcttgcaacggctgctggtgttcgaaggtcgttgagttcccgtcaatcacggcgcacatgttggtgttggaggtgacgatcacgggagtcgggtctatctgggccgaggacttgcatttctggtccacgcgcaccttgcttcctccgagaatggctttggccgactccacgaccttggcggtcatcttcccctcctcccaccagatcaccatcttgtcgacacagtcgttgaagggaaagttctcattggtccagtttacgcacccgtagaagggcacagtgtgggctatggcctccgcgatgttggtcttcccggtagttgcaggcccaaacagccagatggtgttcctcttgccgaactttttcgtggcccatcccagaaagacggaagccgcatattggggatcgtacccgtttagttccaaaattttataaatccgattgctggaaatgtcctccacgggctgctggcccaccaggtagtcgggggcggttttagtcaggctcataatctttcccgcattgtccaaggcagccttgatttgggaccgcgagttggaggccgcattgaaggagatgtatgaggcctggtcctcctggatccactgcttctccgaggtaatccccttgtccacgagccacccgaccagctccatggtggcttcggggccgcggaggctggatcggtcccggtgtcttctatggaggtcaaaacagcgtggatggcgtctccaggcgatctgacggttcactaaacgagctctgcttatatagacctcccaccgtacacgcctaccgcccatttgcgtcaatggggcggagttgttacgacattttggaaagtcccgttgattttggtgccaaaacaaactcccattgacgtcaatggggtggagacttggaaatccccgtgagtcaaaccgctatccacgcccattgatgtactgccaaaaccgcatcaccatggtaatagcgatgactaatacgtagatgtactgccaagtaggaaagtcccataaggtcatgtactgggcataatgccaggcgggccatttaccgtcattgacgtcaatagggggcgtacttggcatatgatacacttgatgtactgccaagtgggcagtttaccgtaaatactccacccattgacgtcaatggaaagtccctattggcgttactatgggaacatacgtcattattgacgtcaatgggcgggggtcgttgggcggtcagccaggcgggccatttaccgtaagttatgtaacgcggaactccatatatgggctatgaactaatgaccccgtaattgattactattaataactagtcaataatcaatgtcttacatccctgggggctttgggggggggctgtccctctagagcggccgccaccgcggtggagctccagcttttgttccctttagtgagggttaattagatcttaatacgactcactatagggcgaattgggtaccgggccccccctcgaggtcgacggtatcgtgtgaaattgttatccgctcacaattccacacaacatacgagccggaagcataaagtgtaaagcctggggtgcctaatgagtgagctaactcacattaattgcgttgcgctcactgcccgctttccagtcgggaaacctgtcgtgccagctgcattaatgaatcggccaacgcgcggggagaggcggtttgcgtattgggcgctcttccgcttcctcgctcactgactcgctgcgctcggtcgttcggctgcggcgagcggtatcagctcactcaaaggcggtaatacggttatccacagaatcaggggataacgcaggaaagaacatgtgagcaaaaggccagcaaaaggccaggaaccgtaaaaaggccgcgttgctggcgtt

SEQ ID NO: 5 - DNA, 11965 bp, synthetic construct
  misc_feature 1..11965: note = plasmid
  source 1..11965: mol_type = other DNA
atgactctcttaaggtagccaaatttccataggctccgcccccctgacgagcatcacaaaaatcgacgctcaagtcagaggtggcgaaacccgacaggactataaagataccaggcgtttccccctggaagctccctcgtgcgctctcctgttccgaccctgccgcttaccggatacctgtccgcctttctcccttcgggaagcgtggcgctttctcatagctcacgctgtaggtatctcagttcggtgtaggtcgttcgctccaagctgggctgtgtgcacgaaccccccgttcagcccgaccgctgcgccttatccggtaactatcgtcttgagtccaacccggtaagacacgacttatcgccactggcagcagccactggtaacaggattagcagagcgaggtatgtaggcggtgctacagagttcttgaagtggtggcctaactacggctacactagaaggacagtatttggtatctgcgctctgctgaagccagttaccttcggaaaaagagttggtagctcttgatccggcaaacaaaccaccgctggtagcggtggtttttttgtttgcaagcagcagattacgcgcagaaaaaaaggatctcaagaagatcctttgatcttttctacggggtctgacgctcagtggaacgaaaactcacgttaagggattttggtcatgagattatcaaaaaggatcttcacctagatccttttaaattaaaaatgaagttttaaatcaatctaaagtatatatgagtaaacttggtctgacagttaccaatgcttaatcagtgaggcacctatctcagcgatctgtctatttcgttcatccatagttgcctgactccccgtcgtgtagataactacgatacgggagggcttaccatctggccccagtgctgcaatgataccgcgagacccacgctcaccggctccagatttatcagcaataaaccagccagccggaagggccgagcgcagaagtggtcctgcaactttatccgcctccatccagtctattaattgttgccgggaagctagagtaagtagttcgccagttaatagtttgcgcaacgttgttgccattgctacaggcatcgtggtgtcacgctcgtcgtttggtatggcttcattcagctccggttcccaacgatcaaggcgagttacatgatcccccatgttgtgcaaaaaagcggttagctccttcggtcctccgatcgttgtcagaagtaagttggccgcagtgttatcactcatggttatggcagcactgcataattctcttactgtcatgccatccgtaagatgcttttctgtgactggtgagtactcaaccaagtcattctgagaatagtgtatgcggcgaccgagttgctcttgcccggcgtcaatacgggataataccgcgccacatagcagaactttaaaagtgctcatcattggaaaacgttcttcggggcgaaaactctcaaggatcttaccgctgttgagatccagttcgatgtaacccactcgtgcacccaactgatcttcagcatcttttactttcaccagcgtttctgggtgagcaaaaacaggaaggcaaaatgccgcaaaaaagggaataagggcgacacggaaatgttgaatactcatactcttcctttttcaatattattgaagcatttatcagggttattgtctcatgagcggatacatatttgaatgtatttagaaaaataaacaaataggggttccgcgcacatttccccgaaaagtgccacctaaattgtaagcgttaatattttgttaaaattcgcgttaaatttttgttaaatcagctcattttttaaccaataggccgaaatcggcaaaatcccttataaatcaaaagaatagaccgagatagggttgagtgttgttccagtttggaacaagagtccactattaaagaacgtggactccaacgtcaaagggcgaaaaaccgtctatcagggcgatggcccactacgtgaaccatcaccctaatcaagttttttggggtcgaggtgccgtaaagcactaaatcggaaccctaaagggagcccccgatttagagcttgacggggaaagccggcgaacgtggcgagaaaggaagggaagaaagcgaaaggagcgggcgctagggcgctggcaagtgtagcggtcacgctgcgcgtaaccaccacacccgccgcgcttaatgcgccgctacagggcgcgtcccattcgccattcaggctgcgcaactgttgggaagggcgatcggtgcgggcctcttcgctattacgccagctggcgaaagggggatgtgctgcaaggcgattaagttgggtaacgccagggttttcccagtcacgacgttgttttatcggtctgtatatcgaggtttatttattaatttgaatagatattaagttttattatatttacacttacatactaataataaattcaacaaacaatttatttatgtttatttatttattaaaaaaaaacaaaaactcaaaatttcttctataaagtaacaaaacttttatcgaattcctgcagcccgggggatccactagttctagagggacagcccccccccaaagcccccagggatgtaattacgtccctcccccgctagggggcagcagcgagccgcccggggctccgctccggtccggcgctccccccgcatccccgagccggcagcgtgcggggacagcccgggcacggggaaggtggcacgggatcgctttcctctgaacgcttctcgctgctctttgagcctgcagacacctggggggatacggggaaaaggcctccaaggccagcttcccacaataagttgggtgaattttggctcattcctcctttctataggattgaggtcagagctttgtgatgggaattctgtggaatgtgtgtcagttagggtgtggaaagtcccgacattgattattgactagttattaatagtaatcaattacggggtcattagttcatagcccatatatggagttccgcgttacataacttacggtaaatggcccgcctggctgaccgcccaacgacccccgcccattgacgtcaataatgacgtatgttcccatagtaacgccaatagggactttccattgacgtcaatgggtggagtatttacggtaaactgcccacttggcagtacatcaagtgtatcatatgccaagtacgccccctattgacgtcaatgacggtaaatggcccgcctggcattatgcccagtacatgaccttatgggactttcctacttggcagtacatctacgtattagtcatcgctattaccatggtgatgcggttttggcagtacatcaatgggcgtggatagcggtttgactcacggggatttccaagtctccaccccattgacgtcaatgggagtttgttttggcaccaaaatcaacgggactttccaaaatgtcgtaacaactccgccccattgacgcaaatgggcggtaggcgtgtacggtgggaggtctatataagcagagctggtttagtgaaccgtcagatcagatctttgtcgatcctaccatccactcgacacacccgccagcggccgcagttgcgcagccatcgacgtcagacgcggaagcttcgatcaactacgcagacaggtaccaaaacaaatgttctcgtcacgtgggcatgaatctgatgctgtttccctgcagacaatgcgagagaatgaatcagaattcaaatatctgcttcactcacggacagaaagactgtttagagtgctttcccgtgtcagaatctcaacccgtttctgtcgtcaaaaaggcgtatcagaaactgtgctacattcatcatatcatgggaaaggtgccagacgcttgcactgcctgcgatctggtcaatgtggatttggatgactgcatctttgaacaataaatgatttaaatcaggtatggctgccgatggttatcttccagattggctcgaggacaacctctctgagggcattcgcgagtggtgggcgctgaaacctggagccccgaagcccaaagccaaccagcaaaagcaggacgacggccggggtctggtgcttcctggctacaagtacctcggacccttcaacggactcgacaagggggagcccgtcaacgcggcggacgcagcggccctcgagcacgacaaggcctacgaccagcagctgcaggcgggtgacaatccgtacctgcggtataaccacgccgacgccgagtttcaggagcgtctgcaagaagatacgtcttttgggggcaacctcgggcgagcagtcttccaggccaagaagcgggttctcgaacctctcggtctggttgaggaaggcgctaagacggctcctggaaagaagagaccggtagagccatcaccccagcgttctccagactcctctacgggcatcggcaagaaaggccaacagcccgccagaaaaagactcaattttggtcagactggcgactcagagtcagttccagaccctcaacctctcggagaacctccagcagcgccctctggtgtgggacctaatacaatggctgcaggcggtggcgcaccaatggcagacaataacgaaggcgccgacggagtgggtagttcctcgggaaattggcattgcgattccacatggctgggcgacagagtcatcaccaccagcacccgaacctgggccctgcccacctacaacaaccacctctacaagcaaatctccaacgggacatcgggaggagccaccaacgacaacacctacttcggctacagcaccccctgggggtattttgactttaacagattccactgccacttttcaccacgtgactggcagcgactcatcaacaacaactggggattccggcccaagagactcagcttcaagctcttcaacatccaggtcaaggaggtcacgcagaatgaaggcaccaagaccatcgccaataacctcaccagcaccatccaggtgtttacggactcggagtaccagctgccgtacgttctcggctctgcccaccagggctgcctgcctccgttcccggcggacgtgttcatgattccccagtacggctacctaacactcaacaacggtagtcaggccgtgggacgctcctccttctactgcctggaatactttccttcgcagatgctgagaaccggcaacaacttccagtttacttacaccttcgaggacgtgcctttccacagcagctacgcccacagccagagcttggaccggctgatgaatcctctgattgaccagtacctgtactacttgtctcggactcaaacaacaggaggcacggcaaatacgcagactctgggcttcagccaaggtgggcctaatacaatggccaatcaggcaaagaactggctgccaggaccctgttaccgccaacaacgcgtctcaacgacaaccgggcaaaacaacaatagcaactttgcctggactgctgggaccaaataccatctgaatggaagaaattcattggctaatcctggcatcgctatggcaacacacaaagacgacgaggagcgtttttttcccagtaacgggatcctgatttttggcaaacaaaatgctgccagagacaatgcggattacagcgatgtcatgctcaccagcgaggaagaaatcaaaaccactaaccctgtggctacagaggaatacggtatcgtggcagataacttgcagcagcaaaacacggctcctcaaattggaactgtcaacagccagggggccttacccggtatggtctggcagaaccgggacgtgtacctgcagggtcccatctgggccaagattcctcacacggacggcaacttccacccgtctccgctgatgggcggctttggcctgaaacatcctccgcctcagatcctgatcaagaacacgcctgtacctgcggatcctccgaccaccttcaaccagtcaaagctgaactctttcatcacgcaatacagcaccggacaggtcagcgtggaaattgaatgggagctgcagaaggaaaacagcaagcgctggaaccccgagatccagtacacctccaactactacaaatctacaagtgtggactttgctgttaatacagaaggcgtgtactctgaaccccgccccattggcacccgttacctcacccgtaatctgtaataacccgggagttctagggatctggcggccgctcgagtctagagggcccgtttaaacccgctgatcagcctcgactgtgccttctagttgccagccatctgttgtttgcccctcccccgtgccttccttgaccctggaaggtgccactcccactgtcctttcctaataaaatgaggaaattgcatcgcattgtctgagtaggtgtcattctattctggggggtggggtggggcaggacagcaagggggaggattgggaagacaatagcaggcatgctggggatgcggtgggctctatgggcgatcgctagcgtttaaacttaagcttggtaccgagctcggatccactagtccagtgtggtggaattcctgcttcgcgatgtacgggccagatatacgcgttgtttactcatgtctgggggtgggcgaagaactccagcatgagatccccgcgctggaggatcatccagccggcgtcccggaaaacgattccgaagcccaacctttgcctgcaggtcgactctagaggatccgaaaaaacctcccacacctccccctgaacctgaaacataaaatgaatgcaattgttgttgttaacttgtttattgcagcttataatggttacaaataaagcaatagcatcacaaatttcacaaataaagcatttttttcactgcattctagttgtggtttgtccaaactcatcaatgtatcttatcatgtctggatccccgcggccgcggtacccacgtgggcgcgccatttaaatgataactcagagagagtgtcctcgagccaatctggaagataaccatcggcagccatacctgatttaaatcatttattgttcaaagatgcagtcatccaaatccacattgaccagatcgcaggcagtgcaagcgtctggcacctttcccatgatatgatgaatgtagcacagtttctgatacgcctttttgacgacagaaacgggttgagattctgacacgggaaagcactctaaacagtctttctgtccgtgagtgaagcagatatttgaattctgattcattctctcgcattgtctgcagggaaacagcatcagattcatgcccacgtgacgagaacatttgttttggtacctgtctgcgtagttgatcgaagcttccgcgtctgacgtcgatggctgcgcaactgactcgcgcacccgtttgggctcacttatatctgcgtcactgggggcgggtcttttcttggctccaccctttttgacgtagaattcatgctccacctcaaccacgtgatcctttgcccaccggaaaaagtctttgacttcctgcttggtgaccttcccaaagtcatgatccagacggcgggtgagttcaaatttgaacatccggtcttgcaacggctgctggtgttcgaaggtcgttgagttcccgtcaatcacggcgcacatgttggtgttggaggtgacgatcacgggagtcgggtctatctgggccgaggacttgcatttctggtccacgcgcaccttgcttcctccgagaatggctttggccgactccacgaccttggcggtcatcttcccctcctcccaccagatcaccatcttgtcgacacagtcgttgaagggaaagttctcattggtccagtttacgcacccgtagaagggcacagtgtgggctatggcctccgcgatgttggtcttcccggtagttgcaggcccaaacagccagatggtgttcctcttgccgaactttttcgtggcccatcccagaaagacggaagccgcatattggggatcgtacccgtttagttccaaaattttataaatccgattgctggaaatgtcctccacgggctgctggcccaccaggtagtcgggggcggttttagtcaggctcataatctttcccgcattgtccaaggcagccttgatttgggaccgcgagttggaggccgcattgaaggagatgtatgaggcctggtcctcctggatccactgcttctccgaggtaatccccttgtccacgagccacccgaccagctccatgtacctggctgaagtttttgatctgatcaccggcgcatcagaattgggattctgattctctttgttctgctcctgcgtctgcgacacgtgcgtcagatgctgcgccaccaaccgtttacgctccgtgagattcaaacaggcgcttaaatactgttccatattagtccacgcccactggagctcaggctgggttttggggagcaagtaattggggatgtagcactcatccaccaccttgttcccgcctccggcgccatttctggtctttgtgaccgcgaaccagtttggcaaagtcggctcgatcccgcggtaaattctctgaatcagtttttcgcgaatctgactcaggaaacgtcccaaaaccatggatttcaccccggtggtttccacgagcacgtgcatgtggaagtagctctctcccttctcaaattgcacaaagaaaagggcctccggggccttactcacacggcgccattccgtcagaaagtcgcgctgcagcttctcggccacggtcaggggtgcctgctcaatcagattcagatccatgtcagaatctggcggcaactcccattccttctcggccacccagttcacaaagctgtcagaaatgccgggcagatgctcgtcaaggtcgctggggaccttaatcacaatctcgtaaaaccccggcatggcggcgataactattatcatcgtgtttttcaaaggaaaaccacgtccccgtggttcggggggcctagacgtttttttaacctcgactaaacacatgtaaagcatgtgcaccgaggccccagatcagatcccatacaatggggtaccttctgggcatccttcagccccttgttgaatacgcttgaggagagccatttgactctttccacaactatccaactcacaacgtggcactggggttgtgccgcctttgcaggtgtatcttatacacgtggcttttggccgcagaggcacctgtcgccaggtggggggttccgctgcctgcaaagggtcgctacagacgttgtttgtcttcaagaagcttccagaggaactgcttccttcacgacattcaacagaccttgcattcctttggcgagaggggaaagacccctaggaatgctcgtcaagaagacagggccaggtttccgggccctcacattgccaaaagacggcaatatggtggaaaataacatatagacaaacgcacaccggccttattccaagcggcttcggccagtaacgttagggggggggggcggaattctatccctcagttatctcagagagagtgtcctcgagccaatctggaagataaccatcggcagccatacctgatttaaatcatttattgttcaaagatgcagtcatccaaatccacattgaccagatcgcaggcagtgcaagcgtctggcacctttcccatgatatgatgaatgtagcacagtttctgatacgcctttttgacgacagaaacgggttgagattctgacacgggaaagcactctaaacagtctttctgtccgtgagtgaagcagatatttgaattctgattcattctctcgcattgtctgcagggaaacagcatcagattcatgcccacgtgacgagaacatttgttttggtacctgtctgcgtagttgatcgaagcttccgcgtctgacgtcgatggctgcgcaactgactcgcgcacccgtttgggctcacttatatctgcgtcactgggggcgggtcttttcttggctccaccctttttgacgtagaattcatgctccacctcaaccacgtgatcctttgcccaccggaaaaagtctttgacttcctgcttggtgaccttcccaaagtcatgatccagacggcgggtgagttcaaatttgaacatccggtcttgcaacggctgctggtgttcgaaggtcgttgagttcccgtcaatcacggcgcacatgttggtgttggaggtgacgatcacgggagtcgggtctatctgggccgaggacttgcatttctggtccacgcgcaccttgcttcctccgagaatggctttggccgactccacgaccttggcggtcatcttcccctcctcccaccagatcaccatcttgtcgacacagtcgttgaagggaaagttctcattggtccagtttacgcacccgtagaagggcacagtgtgggctatggcctccgcgatgttggtcttcccggtagttgcaggcccaaacagccagatggtgttcctcttgccgaactttttcgtggcccatcccagaaagacggaagccgcatattggggatcgtacccgtttagttccaaaattttataaatccgattgctggaaatgtcctccacgggctgctggcccaccaggtagtcgggggcggttttagtcaggctcataatctttcccgcattgtccaaggcagccttgatttgggaccgcgagttggaggccgcattgaaggagatgtatgaggcctggtcctcctggatccactgcttctccgaggtaatccccttgtccacgagccacccgaccagctccatggtggcttcggggccgcggaggctggatcggtcccggtgtcttctatggaggtcaaaacagcgtggatggcgtctccaggcgatctgacggttcactaaacgagctctgcttatatagacctcccaccgtacacgcctaccgcccatttgcgtcaatggggcggagttgttacgacattttggaaagtcccgttgattttggtgccaaaacaaactcccattgacgtcaatggggtggagacttggaaatccccgtgagtcaaaccgctatccacgcccattgatgtactgccaaaaccgcatcaccatggtaatagcgatgactaatacgtagatgtactgccaagtaggaaagtcccataaggtcatgtactgggcataatgccaggcgggccatttaccgtcattgacgtcaatagggggcgtacttggcatatgatacacttgatgtactgccaagtgggcagtttaccgtaaatactccacccattgacgtcaatggaaagtccctattggcgttactatgggaacatacgtcattattgacgtcaatgggcgggggtcgttgggcggtcagccaggcgggccatttaccgtaagttatgtaacgcggaactccatatatgggctatgaactaatgaccccgtaattgattactattaataactagtcaataatcaatgtcttacatccctgggggctttgggggggggctgtccctctagagcggccgccaccgcggtggagctccagcttttgttccctttagtgagggttaattagatcttaatacgactcactatagggcgaattgggtaccgggccccccctcgaggtcgacggtatcgtgtgaaattgttatccgctcacaattccacacaacatacgagccggaagcataaagtgtaaagcctggggtgcctaatgagtgagctaactcacattaattgcgttgcgctcactgcccgctttccagtcgggaaacctgtcgtgccagctgcattaatgaatcggccaacgcgcggggagaggcggtttgcgtattgggcgctcttccgcttcctcgctcactgactcgctgcgctcggtcgttcggctgcggcgagcggtatcagctcactcaaaggcggtaatacggttatccacagaatcaggggataacgcaggaaagaacatgtgagcaaaaggccagcaaaaggccaggaaccgtaaaaaggccgcgttgctggcgtt

SEQ ID NO: 6 - DNA, 8189 bp, synthetic construct
  misc_feature 1..8189: note = plasmid
  source 1..8189: mol_type = other DNA
gcgcgccgatatcgttaacgccccgcgccggccgctctagaactagtggatcccccggaagatcagaagttcctattccgaagttcctattctctagaaagtataggaacttctgatctgcgcagccgccatgccggggttttacgagattgtgattaaggtccccagcgaccttgacgagcatctgcccggcatttctgacagctttgtgaactgggtggccgagaaggaatgggagttgccgccagattctgacatggatctgaatctgattgagcaggcacccctgaccgtggccgagaagctgcagcgcgactttctgacggaatggcgccgtgtgagtaaggccccggaggcccttttctttgtgcaatttgagaagggagagagctacttccacatgcacgtgctcgtggaaaccaccggggtgaaatccatggttttgggacgtttcctgagtcagattcgcgaaaaactgattcagagaatttaccgcgggatcgagccgactttgccaaactggttcgcggtcacaaagaccagaaatggcgccggaggcgggaacaaggtggtggatgagtgctacatccccaattacttgctccccaaaacccagcctgagctccagtgggcgtggactaatatggaacagtatttaagcgcctgtttgaatctcacggagcgtaaacggttggtggcgcagcatctgacgcacgtgtcgcagacgcaggagcagaacaaagagaatcagaatcccaattctgatgcgccggtgatcagatcaaaaacttcagccaggtacatggagctggtcgggtggctcgtggacaaggggattacctcggagaagcagtggatccaggaggaccaggcctcatacatctccttcaatgcggcctccaactcgcggtcccaaatcaaggctgccttggacaatgcgggaaagattatgagcctgactaaaaccgcccccgactacctggtgggccagcagcccgtggaggacatttccagcaatcggatttataaaattttggaactaaacgggtacgatccccaatatgcggcttccgtctttctgggatgggccacgaaaaagttcggcaagaggaacaccatctggctgtttgggcctgcaactaccgggaagaccaacatcgcggaggccatagcccacactgtgcccttctacgggtgcgtaaactggaccaatgagaactttcccttcaacgactgtgtcgacaagatggtgatctggtgggaggaggggaagatgaccgccaaggtcgtggagtcggccaaagccattctcggaggaagcaaggtgcgcgtggaccagaaatgcaagtcctcggcccagatagacccgactcccgtgatcgtcacctccaacaccaacatgtgcgccgtgattgacgggaactcaacgaccttcgaacaccagcagccgttgcaagaccggatgttcaaatttgaactcacccgccgtctggatcatgactttgggaaggtcaccaagcaggaagtcaaagactttttccggtgggcaaaggatcacgtggttgaggtggagcatgaattctacgtcaaaaagggtggagccaagaaaagacccgcccccagtgacgcagatataagtgagcccaaacgggtgcgcgagtcagttgcgcagccatcgacgtcagacgcggaagcttcgatcaactacgcagacaggtaccaaaacaaatgttctcgtcacgtgggcatgaatctgatgctgtttccctgcagacaatgcgagagaatgaatcagaattcaaatatctgcttcactcacggacagaaagactgtttagagtgctttcccgtgtcagaatctcaacccgtttctgtcgtcaaaaaggcgtatcagaaactgtgctacattcatcatatcatgggaaaggtgccagacgcttgcactgcctgcgatctggtcaatgtggatttggatgactgcatctttgaacaataaatgatttaaatcaggtatggctgccgatggttatcttccagattggctcgaggacactctctctgaaggaataagacagtggtggaagctcaaacctggcccaccaccaccaaagcccgcagagcggcataaggacgacagcaggggtcttgtgcttcctgggtacaagtacctcggacccttcaacggactcgacaagggagagccggtcaacgaggcagacgccgcggccctcgagcacgacaaagcctacgaccggcagctcgacagcggagacaacccgtacctcaagtacaaccacgccgacgcggagtttcaggagcgccttaaagaagatacgtcttttgggggcaacctcggacgagcagtcttccaggcgaaaaagagggttcttgaacctctgggcctggttgaggaacctgttaagacggctccgggaaaaaagaggccggtagagcactctcctgtggagccagactcctcctcgggaaccggaaaggcgggccagcagcctgcaagaaaaagattgaattttggtcagactggagacgcagactcagtacctgacccccagcctctcggacagccaccagcagccccctctggtctgggaactaatacgatggctacaggcagtggcgcaccaatggcagacaataacgagggcgccgacggagtgggtaattcctcgggaaattggcattgcgattccacatggatgggcgacagagtcatcaccaccagcacccgaacctgggccctgcccacctacaacaaccacctctacaaacaaatttccagccaatcaggagcctcgaacgacaatcactactttggctacagcaccccttgggggtattttgacttcaacagattccactgccacttttcaccacgtgactggcaaagactcatcaacaacaactggggattccgacccaagagactcaacttcaagctctttaacattcaagtcaaagaggtcacgcagaatgacggtacgacgacgattgccaataaccttaccagcacggttcaggtgtttactgactcggagtaccagctcccgtacgtcctcggctcggcgcatcaaggatgcctcccgccgttcccagcagacgtcttcatggtgccacagtatggatacctcaccctgaacaacgggagtcaggcagtaggacgctcttcattttactgcctggagtactttccttctcagatgctgcgtaccggaaacaactttaccttcagctacacttttgaggacgttcctttccacagcagctacgctcacagccagagtctggaccgtctcatgaatcctctcatcgaccagtacctgtattacttgagcagaacaaacactccaagtggaaccaccacgcagtcaaggcttcagttttctcaggccggagcgagtgacattcgggaccagtctaggaactggcttcctggaccctgttaccgccagcagcgagtatcaaagacatctgcggataacaacaacagtgaatactcgtggactggagctaccaagtaccacctcaatggcagagactctctggtgaatccgggcccggccatggcaagccacaaggacgatgaagaaaagttttttcctcagagcggggttctcatctttgggaagcaaggctcagagaaaacaaatgtggacattgaaaaggtcatgattacagacgaagaggaaatcaggacaaccaatcccgtggctacggagcagtatggttctgtatctaccaacctccagagaggcaacagacaagcagctaccgcagatgtcaacacacaaggcgttcttccaggcatggtctggcaggacagagatgtgtaccttcaggggcccatctgggcaaagattccacacacggacggacattttcacccctctcccctcatgggtggattcggacttaaacaccctcctccacagattctcatcaagaacaccccggtacctgcgaatccttcgaccaccttcagtgcggcaaagtttgcttccttcatcacacagtactccacgggacaggtcagcgtggagatcgagtgggagctgcagaaggaaaacagcaaacgctggaatcccgaaattcagtacacttccaactacaacaagtctgttaatgtggactttactgtggacactaatggcgtgtattcagagcctcgccccattggcaccagatacctgactcgtaatctgtaattgcttgttaatcaataaaccgtttaattcgtttcagttgaactttggtctctgcgtatttctttcttatctagtttccatggctactaaatggcccgcctggctgaccgcccaacgacccccgcccattgacgtcaataatgacgtatgttcccatagtaacgccaatagggactttccattgacgtcaatgggtggagtatttacggtaaactgcccacttggcagtacatcaagtgtatcatatgccaagtacgccccctattgacgtcaatgacggtaaatggcccgcctggcattatgcccagtacatgaccttatgggactttcctacttggcagtacatctacgtattagtcatcgctattaccatggtgatgcggttttggcagtacatcaatgggcgtggatagcggtttgactcacggggatttccaagtctccaccccattgacgtcaatgggagtttgttttggcaccaaaatcaacgggactttccaaaatgtcgtaacaactccgccccattgacgcaaatgggcggtaggcgtgtacggtgggaggtctatataagcagagctggtttagtgaaccggatcctgccattgcatccttctctgcagactaagatggagttcctgaaccaagaccgcttgctggccaacctgtgaaactgggctcaaggtgaggggtgctatctgtgattgagggacatggttaatggaattgtctcacacagaaatcgcacccgtcaccttggcctacttatcaccaccccaaacagaggaacacgccttctccagccacagcctatggaagggccttcagctgctgtggccccgaggtaagcttgggggaggctaactgaaacacggaaggagacaataccggaaggaacccgcgctatgacggcaataaaaagacagaataaaacgcacggtgttgggtcgttgtagataagtagcatggcgggttaatcattaactacagcccgggcgtttaaacagcgggcggaggggtggagtcgtgacgtgaattacgtcatagggttagggaggtcctgtattagaggtcacgtgagtgttttgcgacattttgcgacaccatgtggtctcgctgggggggggggcccgagtgagcacgcagggtctccattttgaagcgggaggtttgaacgagcgctggcgcgctcactggccgtcgttttacaacgtcgtgactgggaaaaccctggcgttacccaacttaatcgccttgcagcacatccccctttcgccagctggcgtaatagcgaagaggcccgcaccgatcgcccttcccaacagttgcgcagcctgaatggcgaatggaaattgtaagcgttaatattttgttaaaattcgcgttaaatttttgttaaatcagctcatttttttaaccaataggccgaaatcggcaaaatcccttataaatcaaaagaatagaccgagatagggttgagtgttgttccagtttggaacaagagtccactattaagaacgtggactccaacgtcaaagggcgaaaaaccgtctatcagggcgatggcccactacgtgaaccatcaccctaatcaagttttttggggtcgaggtgccgtaaagcactaaatcggaaccctaaagggagcccccgatttagagcttgacggggaaagccggcgaacgtggcgagaaaggaagggaagaaagcgaaaggagcgggcgctagggcgctggcaagtgtagcggtcacgctgcgcgtaaccaccacacccgccgcgcttaatgcgccgctacagggcgcgtcaggtggcacttttcggggaaatgtgcgcggaacccctatttgtttatttttctaaatacattcaaatatgtatccgctcatgagacaataaccctgataaatgcttcaataatattgaaaaaggaagagtatgagtattcaacatttccgtgtcgcccttattcccttttttgcggcattttgccttcctgtttttgctcacccagaaacgctggtgaaagtaaaagatgctgaagatcagttgggtgcacgagtgggttacatcgaactggatctcaacagcggtaagatccttgagagttttcgccccgaagaacgttttccaatgatgagcacttttaaagttctgctatgtggcgcggtattatcccgtattgacgccgggcaagagcaactcggtcgccgcatacactattctcagaatgacttggttgagtactcaccagtcacagaaaagcatcttacggatggcatgacagtaagagaattatgcagtgctgccataaccatgagtgataacactgcggccaacttacttctgacaacgatcggaggaccgaaggagctaaccgcttttttgcacaacatgggggatcatgtaactcgccttgatcgttgggaaccggagctgaatgaagccataccaaacgacgagcgtgacaccacgatgcctgtagcaatggcaacaacgttgcgcaaactattaactggcgaactacttactctagcttcccggcaacaattaatagactggatggaggcggataaagttgcaggaccacttctgcgctcggcccttccggctggctggtttattgctgataaatctggagccggtgagcgtgggtctcgcggtatcattgcagcactggggccagatggtaagccctcccgtatcgtagttatctacacgacggggagtcaggcaactatggatgaacgaaatagacagatcgctgagataggtgcctcactgattaagcattggtaactgtcagaccaagtttactcatatatactttagattgatttaaaacttcatttttaatttaaaaggatctaggtgaagatcctttttgataatctcatgaccaaaatcccttaacgtgagttttcgttccactgagcgtcagaccccgtagaaaagatcaaaggatcttcttgagatcctttttttctgcgcgtaatctgctgcttgcaaacaaaaaaaccaccgctaccagcggtggtttgtttgccggatcaagagctaccaactctttttccgaaggtaactggcttcagcagagcgcagataccaaatactgttcttctagtgtagccgtagttaggccaccacttcaagaactctgtagcaccgcctacatacctcgctctgctaatcctgttaccagtggctgctgccagtggcgataagtcgtgtcttaccgggttggactcaagacgatagttaccggataaggcgcagcggtcgggctgaacggggggttcgtgcacacagcccagcttggagcgaacgacctacaccgaactgagatacctacagcgtgagctatgagaaagcgccacgcttcccgaagggagaaaggcggacaggtatccggtaagcggcagggtcggaacaggagagcgcacgagggagcttccagggggaaacgcctggtatctttatagtcctgtcgggtttcgccacctctgacttgagcgtcgatttttgtgatgctcgtcaggggggcggagcctatggaaaaacgccagcaacgcggcctttttacggttcctggccttttgctggccttttgctcacatgttctttcctgcgttatcccctgattctgtggataaccgtattaccgcctttgagtgagctgataccgctcgccgcagccgaacgaccgagcgcagcgagtcagtgagcgaggaagcggaagagcgcccaatacgcaaaccgcctctccccgcgcgttggccgattcattaatgcagctggcacgacaggtttcccgactggaaagcgggcagtgagcgcaacgcaattaatgtgagttagctcactcattaggcaccccaggctttacactttatgcttccggctcgtatgttgtgtggaattgtgagcggataacaatttcacacaggaaacagctatgaccatgattacgccaa

SEQ ID NO: 7 - DNA, 7294 bp, synthetic construct
  misc_feature 1..7294: note = plasmid
  source 1..7294: mol_type = other DNA
gcgcgccgatatcgttaacgccccgcgccggccgctctagaactagtggatcccccggaagatcagaagttcctattccgaagttcctattctctagaaagtataggaacttctgatctgcgcagccgccatgccggggttttacgagattgtgattaaggtccccagcgaccttgacgagcatctgcccggcatttctgacagctttgtgaactgggtggccgagaaggaatgggagttgccgccagattctgacatggatctgaatctgattgagcaggcacccctgaccgtggccgagaagctgcagcgcgactttctgacggaatggcgccgtgtgagtaaggccccggaggcccttttctttgtgcaatttgagaagggagagagctacttccacatgcacgtgctcgtggaaaccaccggggtgaaatccatggttttgggacgtttcctgagtcagattcgcgaaaaactgattcagagaatttaccgcgggatcgagccgactttgccaaactggttcgcggtcacaaagaccagaaatggcgccggaggcgggaacaaggtggtggatgagtgctacatccccaattacttgctccccaaaacccagcctgagctccagtgggcgtggactaatatggaacagtatttaagcgcctgtttgaatctcacggagcgtaaacggttggtggcgcagcatctgacgcacgtgtcgcagacgcaggagcagaacaaagagaatcagaatcccaattctgatgcgccggtgatcagatcaaaaacttcagccaggtacatggagctggtcgggtggctcgtggacaaggggattacctcggagaagcagtggatccaggaggaccaggcctcatacatctccttcaatgcggcctccaactcgcggtcccaaatcaaggctgccttggacaatgcgggaaagattatgagcctgactaaaaccgcccccgactacctggtgggccagcagcccgtggaggacatttccagcaatcggatttataaaattttggaactaaacgggtacgatccccaatatgcggcttccgtctttctgggatgggccacgaaaaagttcggcaagaggaacaccatctggctgtttgggcctgcaactaccgggaagaccaacatcgcggaggccatagcccacactgtgcccttctacgggtgcgtaaactggaccaatgagaactttcccttcaacgactgtgtcgacaagatggtgatctggtgggaggaggggaagatgaccgccaaggtcgtggagtcggccaaagccattctcggaggaagcaaggtgcgcgtggaccagaaatgcaagtcctcggcccagatagacccgactcccgtgatcgtcacctccaacaccaacatgtgcgccgtgattgacgggaactcaacgaccttcgaacaccagcagccgttgcaagaccggatgttcaaatttgaactcacccgccgtctggatcatgactttgggaaggtcaccaagcaggaagtcaaagactttttccggtgggcaaaggatcacgtggttgaggtggagcatgaattctacgtcaaaaagggtggagccaagaaaagacccgcccccagtgacgcagatataagtgagcccaaacgggtgcgcgagtcagttgcgcagccatcgacgtcagacgcggaagcttcgatcaactacgcagacaggtaccaaaacaaatgttctcgtcacgtgggcatgaatctgatgctgtttccctgcagacaatgcgagagaatgaatcagaattcaaatatctgcttcactcacggacagaaagactgtttagagtgctttcccgtgtcagaatctcaacccgtttctgtcgtcaaaaaggcgtatcagaaactgtgctacattcatcatatcatgggaaaggtgccagacgcttgcactgcctgcgatctggtcaatgtggatttggatgactgcatctttgaacaataaatgatttaaatcaggtatgtcttttgttgatcaccctccagattggttggaagaagttggtgaaggtcttcgcgagtttttgggccttgaagcgggcccaccgaaaccaaaacccaatcagcagcatcaagatcaagcccgtggtcttgtgctgcctggttataactatctcggacccggaaacggtctcgatcgaggagagcctgtcaacagggcagacgaggtcgcgcgagagcacgacatctcgtacaacgagcagcttgaggcgggagacaacccctacctcaagtacaaccacgcggacgccgagtttcaggagaagctcgccgacgacacatccttcgggggaaacctcggaaaggcagtctttcaggccaagaaaagggttctcgaaccttttggcctggttgaagagggtgctaagacggcccctaccggaaagcggatagacgaccactttccaaaaagaaagaaggctcggaccgaagaggactccaagccttccacctcgtcagacgccgaagctggacccagcggatcccagcagctgcaaatcccagcccaaccagcctcaagtttgggagctgatacaatgtctgcgggaggtggcggcccattgggcgacaataaccaaggtgccgatggagtgggcaatgcctcgggagattggcattgcgattccacgtggatgggggacagagtcgtcaccaagtccacccgaacctgggtgctgcccagctacaacaaccaccagtaccgagagatcaaaagcggctccgtcgacggaagcaacgccaacgcctactttggatacagcaccccctgggggtactttgactttaaccgcttccacagccactggagcccccgagactggcaaagactcatcaacaactactggggcttcagaccccggtccctcagagtcaaaatcttcaacattcaagtcaaagaggtcacggtgcaggactccaccaccaccatcgccaacaacctcacctccaccgtccaagtgtttacggacgacgactaccagctgccctacgtcgtcggcaacgggaccgagggatgcctgccggccttccctccgcaggtctttacgctgccgcagtacggttacgcgacgctgaaccgcgacaacacagaaaatcccaccgagaggagcagcttcttctgcctagagtactttcccagcaagatgctgagaacgggcaacaactttgagtttacctacaactttgaggaggtgcccttccactccagcttcgctcccagtcagaacctgttcaagctggccaacccgctggtggaccagtacttgtaccgcttcgtgagcacaaataacactggcggagtccagttcaacaagaacctggccgggagatacgccaacacctacaaaaactggttcccggggcccatgggccgaacccagggctggaacctgggctccggggtcaaccgcgccagtgtcagcgccttcgccacgaccaataggatggagctcgagggcgcgagttaccaggtgcccccgcagccgaacggcatgaccaacaacctccagggcagcaacacctatgccctggagaacactatgatcttcaacagccagccggcgaacccgggcaccaccgccacgtacctcgagggcaacatgctcatcaccagcgagagcgagacgcagccggtgaaccgcgtggcgtacaacgtcggcgggcagatggccaccaacaaccagagctccaccactgcccccgcgaccggcacgtacaacctccaggaaatcgtgcccggcagcgtgtggatggagagggacgtgtacctccaaggacccatctgggccaagatcccagagacgggggcgcactttcacccctctccggccatgggcggattcggactcaaacacccaccgcccatgatgctcatcaagaacacgcctgtgcccggaaatatcaccagcttctcggacgtgcccgtcagcagcttcatcacccagtacagcaccgggcaggtcaccgtggagatggagtgggagctcaagaaggaaaactccaagaggtggaacccagagatccagtacacaaacaactacaacgacccccagtttgtggactttgccccggacagcaccggggaatacagaaccaccagacctatcggaacccgataccttacccgacccctttaattgcttgttaatcaataaaccgtttaattcgtttcagttgaactttggtctctgcgtatttctttcttatctagtttccatggctacgtagataagtagcatggcgggttaatcattaactacagcccgggcgtttaaacagcgggcggaggggtggagtcgtgacgtgaattacgtcatagggttagggaggtcctgtattagaggtcacgtgagtgttttgcgacattttgcgacaccatgtggtctcgctgggggggggggcccgagtgagcacgcagggtctccattttgaagcgggaggtttgaacgagcgctggcgcgctcactggccgtcgttttacaacgtcgtgactgggaaaaccctggcgttacccaacttaatcgccttgcagcacatccccctttcgccagctggcgtaatagcgaagaggcccgcaccgatcgcccttcccaacagttgcgcagcctgaatggcgaatggaaattgtaagcgttaatattttgttaaaattcgcgttaaatttttgttaaatcagctcatttttttaaccaataggccgaaatcggcaaaatcccttataaatcaaaagaatagaccgagatagggttgagtgttgttccagtttggaacaagagtccactattaagaacgtggactccaacgtcaaagggcgaaaaaccgtctatcagggcgatggcccactacgtgaaccatcaccctaatcaagttttttggggtcgaggtgccgtaaagcactaaatcggaaccctaaagggagcccccgatttagagcttgacggggaaagccggcgaacgtggcgagaaaggaagggaagaaagcgaaaggagcgggcgctagggcgctggcaagtgtagcggtcacgctgcgcgtaaccaccacacccgccgcgcttaatgcgccgctacagggcgcgtcaggtggcacttttcggggaaatgtgcgcggaacccctatttgtttatttttctaaatacattcaaatatgtatccgctcatgagacaataaccctgataaatgcttcaataatattgaaaaaggaagagtatgagtattcaacatttccgtgtcgcccttattcccttttttgcggcattttgccttcctgtttttgctcacccagaaacgctggtgaaagtaaaagatgctgaagatcagttgggtgcacgagtgggttacatcgaactggatctcaacagcggtaagatccttgagagttttcgccccgaagaacgttttccaatgatgagcacttttaaagttctgctatgtggcgcggtattatcccgtattgacgccgggcaagagcaactcggtcgccgcatacactattctcagaatgacttggttgagtactcaccagtcacagaaaagcatcttacggatggcatgacagtaagagaattatgcagtgctgccataaccatgagtgataacactgcggccaacttacttctgacaacgatcggaggaccgaaggagctaaccgcttttttgcacaacatgggggatcatgtaactcgccttgatcgttgggaaccggagctgaatgaagccataccaaacgacgagcgtgacaccacgatgcctgtagcaatggcaacaacgttgcgcaaactattaactggcgaactacttactctagcttcccggcaacaattaatagactggatggaggcggataaagttgcaggaccacttctgcgctcggcccttccggctggctggtttattgctgataaatctggagccggtgagcgtgggtctcgcggtatcattgcagcactggggccagatggtaagccctcccgtatcgtagttatctacacgacggggagtcaggcaactatggatgaacgaaatagacagatcgctgagataggtgcctcactgattaagcattggtaactgtcagaccaagtttactcatatatactttagattgatttaaaacttcatttttaatttaaaaggatctaggtgaagatcctttttgataatctcatgaccaaaatcccttaacgtgagttttcgttccactgagcgtcagaccccgtagaaaagatcaaaggatcttcttgagatcctttttttctgcgcgtaatctgctgcttgcaaacaaaaaaaccaccgctaccagcggtggtttgtttgccggatcaagagctaccaactctttttccgaaggtaactggcttcagcagagcgcagataccaaatactgttcttctagtgtagccgtagttaggccaccacttcaagaactctgtagcaccgcctacatacctcgctctgctaatcctgttaccagtggctgctgccagtggcgataagtcgtgtcttaccgggttggactcaagacgatagttaccggataaggcgcagcggtcgggctgaacggggggttcgtgcacacagcccagcttggagcgaacgacctacaccgaactgagatacctacagcgtgagctatgagaaagcgccacgcttcccgaagggagaaaggcggacaggtatccggtaagcggcagggtcggaacaggagagcgcacgagggagcttccagggggaaacgcctggtatctttatagtcctgtcgggtttcgccacctctgacttgagcgtcgatttttgtgatgctcgtcaggggggcggagcctatggaaaaacgccagcaacgcggcctttttacggttcctggccttttgctggccttttgctcacatgttctttcctgcgttatcccctgattctgtggataaccgtattaccgcctttgagtgagctgataccgctcgccgcagccgaacgaccgagcgcagcgagtcagtgagcgaggaagcggaagagcgcccaatacgcaaaccgcctctccccgcgcgttggccgattcattaatgcagctggcacgacaggtttcccgactggaaagcgggcagtgagcgcaacgcaattaatgtgagttagctcactcattaggcaccccaggctttacactttatgcttccggctcgtatgttgtgtggaattgtgagcggataacaatttcacacaggaaacagctatgaccatgattacgccaa

SEQ ID NO: 8 - DNA, 7330 bp, synthetic construct
  misc_feature 1..7330: note = plasmid
  source 1..7330: mol_type = other DNA
gcgcgccgatatcgttaacgccccgcgccggccgctctagaactagtggatcccccggaagatcagaagttcctattccgaagttcctattctctagaaagtataggaacttctgatctgcgcagccgccatgccggggttttacgagattgtgattaaggtccccagcgaccttgacgagcatctgcccggcatttctgacagctttgtgaactgggtggccgagaaggaatgggagttgccgccagattctgacatggatctgaatctgattgagcaggcacccctgaccgtggccgagaagctgcagcgcgactttctgacggaatggcgccgtgtgagtaaggccccggaggcccttttctttgtgcaatttgagaagggagagagctacttccacatgcacgtgctcgtggaaaccaccggggtgaaatccatggttttgggacgtttcctgagtcagattcgcgaaaaactgattcagagaatttaccgcgggatcgagccgactttgccaaactggttcgcggtcacaaagaccagaaatggcgccggaggcgggaacaaggtggtggatgagtgctacatccccaattacttgctccccaaaacccagcctgagctccagtgggcgtggactaatatggaacagtatttaagcgcctgtttgaatctcacggagcgtaaacggttggtggcgcagcatctgacgcacgtgtcgcagacgcaggagcagaacaaagagaatcagaatcccaattctgatgcgccggtgatcagatcaaaaacttcagccaggtacatggagctggtcgggtggctcgtggacaaggggattacctcggagaagcagtggatccaggaggaccaggcctcatacatctccttcaatgcggcctccaactcgcggtcccaaatcaaggctgccttggacaatgcgggaaagattatgagcctgactaaaaccgcccccgactacctggtgggccagcagcccgtggaggacatttccagcaatcggatttataaaattttggaactaaacgggtacgatccccaatatgcggcttccgtctttctgggatgggccacgaaaaagttcggcaagaggaacaccatctggctgtttgggcctgcaactaccgggaagaccaacatcgcggaggccatagcccacactgtgcccttctacgggtgcgtaaactggaccaatgagaactttcccttcaacgactgtgtcgacaagatggtgatctggtgggaggaggggaagatgaccgccaaggtcgtggagtcggccaaagccattctcggaggaagcaaggtgcgcgtggaccagaaatgcaagtcctcggcccagatagacccgactcccgtgatcgtcacctccaacaccaacatgtgcgccgtgattgacgggaactcaacgaccttcgaacaccagcagccgttgcaagaccggatgttcaaatttgaactcacccgccgtctggatcatgactttgggaaggtcaccaagcaggaagtcaaagactttttccggtgggcaaaggatcacgtggttgaggtggagcatgaattctacgtcaaaaagggtggagccaagaaaagacccgcccccagtgacgcagatataagtgagcccaaacgggtgcgcgagtcagttgcgcagccatcgacgtcagacgcggaagcttcgatcaactacgcagacaggtaccaaaacaaatgttctcgtcacgtgggcatgaatctgatgctgtttccctgcagacaatgcgagagaatgaatcagaattcaaatatctgcttcactcacggacagaaagactgtttagagtgctttcccgtgtcagaatctcaacccgtttctgtcgtcaaaaaggcgtatcagaaactgtgctacattcatcatatcatgggaaaggtgccagacgcttgcactgcctgcgatctggtcaatgtggatttggatgactgcatctttgaacaataaatgatttaaatcaggtatggctgccgatggttatcttccagattggctcgaggacaacctctctgagggcattcgcgagtggtgggacttgaaacctggagccccgaaacccaaagccaaccagcaaaagcaggacgacggccggggtctggtgcttcctggctacaagtacctcggacccttcaacggactcgacaagggggagcccgtcaacgcggcggatgcagcggccctcgagcacgacaaggcctacgaccagcagctcaaagcgggtgacaatccgtacctgcggtataaccacgccgacgccgagtttcaggagcgtctgcaagaagatacgtcttttgggggcaacctcgggcgagcagtcttccaggccaagaagagggttctcgaaccttttggtctggttgaggaaggtgctaagacggctcctggaaagaaacgtccggtagagcagtcgccacaagagccagactcctcctcgggcattggcaagacaggccagcagcccgctaaaaagagactcaattttggtcagactggcgactcagagtcagtccccgacccacaacctctcggagaacctccagcaacccccgctgctgtgggacctactacaatggcttcaggcggtggcgcaccaatggcagacaataacgaaggcgccgacggagtgggtaatgcctcaggaaattggcattgcgattccacatggctgggcgacagagtcatcaccaccagcacccgaacatgggccttgcccacctataacaaccacctctacaagcaaatctccagtgcttcaacgggggccagcaacgacaaccactacttcggctacagcaccccctgggggtattttgatttcaacagattccactgccatttctcaccacgtgactggcagcgactcatcaacaacaattggggattccggcccaagagactcaacttcaagctcttcaacatccaagtcaaggaggtcacgacgaatgatggcgtcacgaccatcgctaataaccttaccagcacggttcaagtcttctcggactcggagtaccagttgccgtacgtcctcggctctgcgcaccagggctgcctccctccgttcccggcggacgtgttcatgattccgcagtacggctacctaacgctcaacaatggcagccaggcagtgggacggtcatccttttactgcctggaatatttcccatcgcagatgctgagaacgggcaataactttaccttcagctacaccttcgaggacgtgcctttccacagcagctacgcgcacagccagagcctggaccggctgatgaatcctctcatcgaccagtacctgtattacctgaacagaactcagaatcagtccggaagtgcccaaaacaaggacttgctgtttagccgggggtctccagctggcatgtctgttcagcccaaaaactggctacctggaccctgttaccggcagcagcgcgtttctaaaacaaaaacagacaacaacaacagcaactttacctggactggtgcttcaaaatataaccttaatgggcgtgaatctataatcaaccctggcactgctatggcctcacacaaagacgacaaagacaagttctttcccatgagcggtgtcatgatttttggaaaggagagcgccggagcttcaaacactgcattggacaatgtcatgatcacagacgaagaggaaatcaaagccactaaccccgtggccaccgaaagatttgggactgtggcagtcaatctccagagcagcagcacagaccctgcgaccggagatgtgcatgttatgggagccttacctggaatggtgtggcaagacagagacgtatacctgcagggtcctatttgggccaaaattcctcacacggatggacactttcacccgtctcctctcatgggcggctttggacttaagcacccgcctcctcagatcctcatcaaaaacacgcctgttcctgcgaatcctccggcagagttttcggctacaaagtttgcttcattcatcacccagtattccacaggacaagtgagcgtggagattgaatgggagctgcagaaagaaaacagcaaacgctggaatcccgaagtgcagtatacatctaactatgcaaaatctgccaacgttgatttcactgtggacaacaatggactttatactgagcctcgccccattggcacccgttacctcacccgtcccctgtaattgcttgttaatcaataaaccgtttaattcgtttcagttgaactttggtctctgcgtatttctttcttatctagtttccatggctacgtagataagtagcatggcgggttaatcattaactacagcccgggcgtttaaacagcgggcggaggggtggagtcgtgacgtgaattacgtcatagggttagggaggtcctgtattagaggtcacgtgagtgttttgcgacattttgcgacaccatgtggtctcgctgggggggggggcccgagtgagcacgcagggtctccattttgaagcgggaggtttgaacgagcgctggcgcgctcactggccgtcgttttacaacgtcgtgactgggaaaaccctggcgttacccaacttaatcgccttgcagcacatccccctttcgccagctggcgtaatagcgaagaggcccgcaccgatcgcccttcccaacagttgcgcagcctgaatggcgaatggaaattgtaagcgttaatattttgttaaaattcgcgttaaatttttgttaaatcagctcatttttttaaccaataggccgaaatcggcaaaatcccttataaatcaaaagaatagaccgagatagggttgagtgttgttccagtttggaacaagagtccactattaagaacgtggactccaacgtcaaagggcgaaaaaccgtctatcagggcgatggcccactacgtgaaccatcaccctaatcaagttttttggggtcgaggtgccgtaaagcactaaatcggaaccctaaagggagcccccgatttagagcttgacggggaaagccggcgaacgtggcgagaaaggaagggaagaaagcgaaaggagcgggcgctagggcgctggcaagtgtagcggtcacgctgcgcgtaaccaccacacccgccgcgcttaatgcgccgctacagggcgcgtcaggtggcacttttcggggaaatgtgcgcggaacccctatttgtttatttttctaaatacattcaaatatgtatccgctcatgagacaataaccctgataaatgcttcaataatattgaaaaaggaagagtatgagtattcaacatttccgtgtcgcccttattcccttttttgcggcattttgccttcctgtttttgctcacccagaaacgctggtgaaagtaaaagatgctgaagatcagttgggtgcacgagtgggttacatcgaactggatctcaacagcggtaagatccttgagagttttcgccccgaagaacgttttccaatgatgagcacttttaaagttctgctatgtggcgcggtattatcccgtattgacgccgggcaagagcaactcggtcgccgcatacactattctcagaatgacttggttgagtactcaccagtcacagaaaagcatcttacggatggcatgacagtaagagaattatgcagtgctgccataaccatgagtgataacactgcggccaacttacttctgacaacgatcggaggaccgaaggagctaaccgcttttttgcacaacatgggggatcatgtaactcgccttgatcgttgggaaccggagctgaatgaagccataccaaacgacgagcgtgacaccacgatgcctgtagcaatggcaacaacgttgcgcaaactattaactggcgaactacttactctagcttcccggcaacaattaatagactggatggaggcggataaagttgcaggaccacttctgcgctcggcccttccggctggctggtttattgctgataaatctggagccggtgagcgtgggtctcgcggtatcattgcagcactggggccagatggtaagccctcccgtatcgtagttatctacacgacggggagtcaggcaactatggatgaacgaaatagacagatcgctgagataggtgcctcactgattaagcattggtaactgtcagaccaagtttactcatatatactttagattgatttaaaacttcatttttaatttaaaaggatctaggtgaagatcctttttgataatctcatgaccaaaatcccttaacgtgagttttcgttccactgagcgtcagaccccgtagaaaagatcaaaggatcttcttgagatcctttttttctgcgcgtaatctgctgcttgcaaacaaaaaaaccaccgctaccagcggtggtttgtttgccggatcaagagctaccaactctttttccgaaggtaactggcttcagcagagcgcagataccaaatactgttcttctagtgtagccgtagttaggccaccacttcaagaactctgtagcaccgcctacatacctcgctctgctaatcctgttaccagtggctgctgccagtggcgataagtcgtgtcttaccgggttggactcaagacgatagttaccggataaggcgcagcggtcgggctgaacggggggttcgtgcacacagcccagcttggagcgaacgacctacaccgaactgagatacctacagcgtgagctatgagaaagcgccacgcttcccgaagggagaaaggcggacaggtatccggtaagcggcagggtcggaacaggagagcgcacgagggagcttccagggggaaacgcctggtatctttatagtcctgtcgggtttcgccacctctgacttgagcgtcgatttttgtgatgctcgtcaggggggcggagcctatggaaaaacgccagcaacgcggcctttttacggttcctggccttttgctggccttttgctcacatgttctttcctgcgttatcccctgattctgtggataaccgtattaccgcctttgagtgagctgataccgctcgccgcagccgaacgaccgagcgcagcgagtcagtgagcgaggaagcggaagagcgcccaatacgcaaaccgcctctccccgcgcgttggccgattcattaatgcagctggcacgacaggtttcccgactggaaagcgggcagtgagcgcaacgcaattaatgtgagttagctcactcattaggcaccccaggctttacactttatgcttccggctcgtatgttgtgtggaattgtgagcggataacaatttcacacaggaaacagctatgaccatgattacgccaa

SEQ ID NO: 9 - DNA, 7336 bp, synthetic construct
  misc_feature 1..7336: note = plasmid
  source 1..7336: mol_type = other DNA
cttattcccttttttgcggcattttgccttcctgtttttgctcacccagaaacgctggtgaaagtaaaagatgctgaagatcagttgggtgcacgagtgggttacatcgaactggatctcaacagcggtaagatccttgagagttttcgccccgaagaacgttttccaatgatgagcacttttaaagttctgctatgtggcgcggtattatcccgtattgacgccgggcaagagcaactcggtcgccgcatacactattctcagaatgacttggttgagtactcaccagtcacagaaaagcatcttacggatggcatgacagtaagagaattatgcagtgctgccataaccatgagtgataacactgcggccaacttacttctgacaacgatcggaggaccgaaggagctaaccgcttttttgcacaacatgggggatcatgtaactcgccttgatcgttgggaaccggagctgaatgaagccataccaaacgacgagcgtgacaccacgatgcctgtagcaatggcaacaacgttgcgcaaactattaactggcgaactacttactctagcttcccggcaacaattaatagactggatggaggcggataaagttgcaggaccacttctgcgctcggcccttccggctggctggtttattgctgataaatctggagccggtgagcgtgggtctcgcggtatcattgcagcactggggccagatggtaagccctcccgtatcgtagttatctacacgacggggagtcaggcaactatggatgaacgaaatagacagatcgctgagataggtgcctcactgattaagcattggtaactgtcagaccaagtttactcatatatactttagattgatttaaaacttcatttttaatttaaaaggatctaggtgaagatcctttttgataatctcatgaccaaaatcccttaacgtgagttttcgttccactgagcgtcagaccccgtagaaaagatcaaaggatcttcttgagatcctttttttctgcgcgtaatctgctgcttgcaaacaaaaaaaccaccgctaccagcggtggtttgtttgccggatcaagagctaccaactctttttccgaaggtaactggcttcagcagagcgcagataccaaatactgttcttctagtgtagccgtagttaggccaccacttcaagaactctgtagcaccgcctacatacctcgctctgctaatcctgttaccagtggctgctgccagtggcgataagtcgtgtcttaccgggttggactcaagacgatagttaccggataaggcgcagcggtcgggctgaacggggggttcgtgcacacagcccagcttggagcgaacgacctacaccgaactgagatacctacagcgtgagctatgagaaagcgccacgcttcccgaagggagaaaggcggacaggtatccggtaagcggcagggtcggaacaggagagcgcacgagggagcttccagggggaaacgcctggtatctttatagtcctgtcgggtttcgccacctctgacttgagcgtcgatttttgtgatgctcgtcaggggggcggagcctatggaaaaacgccagcaacgcggcctttttacggttcctggccttttgctggccttttgctcacatgttctttcctgcgttatcccctgattctgtggataaccgtattaccgcctttgagtgagctgataccgctcgccgcagccgaacgaccgagcgcagcgagtcagtgagcgaggaagcggaagagcgcccaatacgcaaaccgcctctccccgcgcgttggccgattcattaatgcagctggcacgacaggtttcccgactggaaagcgggcagtgagcgcaacgcaattaatgtgagttagctcactcattaggcaccccaggctttacactttatgcttccggctcgtatgttgtgtggaattgtgagcggataacaatttcacacaggaaacagctatgaccatgattacgccaagcgcgccgatatcgttaacgccccgcgccggccgctctagaactagtggatcccccggaagatcagaagttcctattccgaagttcctattctctagaaagtataggaacttctgatctgcgcagccgccatgccggggttttacgagattgtgattaaggtccccagcgaccttgacgagcatctgcccggcatttctgacagctttgtgaactgggtggccgagaaggaatgggagttgccgccagattctgacatggatctgaatctgattgagcaggcacccctgaccgtggccgagaagctgcagcgcgactttctgacggaatggcgccgtgtgagtaaggccccggaggcccttttctttgtgcaatttgagaagggagagagctacttccacatgcacgtgctcgtggaaaccaccggggtgaaatccatggttttgggacgtttcctgagtcagattcgcgaaaaactgattcagagaatttaccgcgggatcgagccgactttgccaaactggttcgcggtcacaaagaccagaaatggcgccggaggcgggaacaaggtggtggatgagtgctacatccccaattacttgctccccaaaacccagcctgagctccagtgggcgtggactaatatggaacagtatttaagcgcctgtttgaatctcacggagcgtaaacggttggtggcgcagcatctgacgcacgtgtcgcagacgcaggagcagaacaaagagaatcagaatcccaattctgatgcgccggtgatcagatcaaaaacttcagccaggtacatggagctggtcgggtggctcgtggacaaggggattacctcggagaagcagtggatccaggaggaccaggcctcatacatctccttcaatgcggcctccaactcgcggtcccaaatcaaggctgccttggacaatgcgggaaagattatgagcctgactaaaaccgcccccgactacctggtgggccagcagcccgtggaggacatttccagcaatcggatttataaaattttggaactaaacgggtacgatccccaatatgcggcttccgtctttctgggatgggccacgaaaaagttcggcaagaggaacaccatctggctgtttgggcctgcaactaccgggaagaccaacatcgcggaggccatagcccacactgtgcccttctacgggtgcgtaaactggaccaatgagaactttcccttcaacgactgtgtcgacaagatggtgatctggtgggaggaggggaagatgaccgccaaggtcgtggagtcggccaaagccattctcggaggaagcaaggtgcgcgtggaccagaaatgcaagtcctcggcccagatagacccgactcccgtgatcgtcacctccaacaccaacatgtgcgccgtgattgacgggaactcaacgaccttcgaacaccagcagccgttgcaagaccggatgttcaaatttgaactcacccgccgtctggatcatgactttgggaaggtcaccaagcaggaagtcaaagactttttccggtgggcaaaggatcacgtggttgaggtggagcatgaattctacgtcaaaaagggtggagccaagaaaagacccgcccccagtgacgcagatataagtgagcccaaacgggtgcgcgagtcagttgcgcagccatcgacgtcagacgcggaagcttcgatcaactacgcagacaggtaccaaaacaaatgttctcgtcacgtgggcatgaatctgatgctgtttccctgcagacaatgcgagagaatgaatcagaattcaaatatctgcttcactcacggacagaaagactgtttagagtgctttcccgtgtcagaatctcaacccgtttctgtcgtcaaaaaggcgtatcagaaactgtgctacattcatcatatcatgggaaaggtgccagacgcttgcactgcctgcgatctggtcaatgtggatttggatgactgcatctttgaacaataaatgatttaaatcaggtatggctgccgatggttatcttccagattggctcgaggacaacctctctgagggcattcgcgagtggtgggcgctgaaacctggagccccgaagcccaaagccaaccagcaaaagcaggacgacggccggggtctggtgcttcctggctacaagtacctcggacccttcaacggactcgacaagggggagcccgtcaacgcggcggacgcagcggccctcgagcacgacaaggcctacgaccagcagctgcaggcgggtgacaatccgtacctgcggtataaccacgccgacgccgagtttcaggagcgtctgcaagaagatacgtcttttgggggcaacctcgggcgagcagtcttccaggccaagaagcgggttctcgaacctctcggtctggttgaggaaggcgctaagacggctcctggaaagaagagaccggtagagccatcaccccagcgttctccagactcctctacgggcatcggcaagaaaggccaacagcccgccagaaaaagactcaattttggtcagactggcgactcagagtcagttccagaccctcaacctctcggagaacctccagcagcgccctctggtgtgggacctaatacaatggctgcaggcggtggcgcaccaatggcagacaataacgaaggcgccgacggagtgggtagttcctcgggaaattggcattgcgattccacatggctgggcgacagagtcatcaccaccagcacccgaacctgggccctgcccacctacaacaaccacctctacaagcaaatctccaacgggacatcgggaggagccaccaacgacaacacctacttcggctacagcaccccctgggggtattttgactttaacagattccactgccacttttcaccacgtgactggcagcgactcatcaacaacaactggggattccggcccaagagactcagcttcaagctcttcaacatccaggtcaaggaggtcacgcagaatgaaggcaccaagaccatcgccaataacctcaccagcaccatccaggtgtttacggactcggagtaccagctgccgtacgttctcggctctgcccaccagggctgcctgcctccgttcccggcggacgtgttcatgattccccagtacggctacctaacactcaacaacggtagtcaggccgtgggacgctcctccttctactgcctggaatactttccttcgcagatgctgagaaccggcaacaacttccagtttacttacaccttcgaggacgtgcctttccacagcagctacgcccacagccagagcttggaccggctgatgaatcctctgattgaccagtacctgtactacttgtctcggactcaaacaacaggaggcacggcaaatacgcagactctgggcttcagccaaggtgggcctaatacaatggccaatcaggcaaagaactggctgccaggaccctgttaccgccaacaacgcgtctcaacgacaaccgggcaaaacaacaatagcaactttgcctggactgctgggaccaaataccatctgaatggaagaaattcattggctaatcctggcatcgctatggcaacacacaaagacgacgaggagcgtttttttcccagtaacgggatcctgatttttggcaaacaaaatgctgccagagacaatgcggattacagcgatgtcatgctcaccagcgaggaagaaatcaaaaccactaaccctgtggctacagaggaatacggtatcgtggcagataacttgcagcagcaaaacacggctcctcaaattggaactgtcaacagccagggggccttacccggtatggtctggcagaaccgggacgtgtacctgcagggtcccatctgggccaagattcctcacacggacggcaacttccacccgtctccgctgatgggcggctttggcctgaaacatcctccgcctcagatcctgatcaagaacacgcctgtacctgcggatcctccgaccaccttcaaccagtcaaagctgaactctttcatcacgcaatacagcaccggacaggtcagcgtggaaattgaatgggagctgcagaaggaaaacagcaagcgctggaaccccgagatccagtacacctccaactactacaaatctacaagtgtggactttgctgttaatacagaaggcgtgtactctgaaccccgccccattggcacccgttacctcacccgtaatctgtaattgcttgttaatcaataaaccgtttaattcgtttcagttgaactttggtctctgcgtatttctttcttatctagtttccatggctacgtagataagtagcatggcgggttaatcattaactacagcccgggcgtttaaacagcgggcggaggggtggagtcgtgacgtgaattacgtcatagggttagggaggtcctgtattagaggtcacgtgagtgttttgcgacattttgcgacaccatgtggtctcgctgggggggggggcccgagtgagcacgcagggtctccattttgaagcgggaggtttgaacgagcgctggcgcgctcactggccgtcgttttacaacgtcgtgactgggaaaaccctggcgttacccaacttaatcgccttgcagcacatccccctttcgccagctggcgtaatagcgaagaggcccgcaccgatcgcccttcccaacagttgcgcagcctgaatggcgaatggaaattgtaagcgttaatattttgttaaaattcgcgttaaatttttgttaaatcagctcatttttttaaccaataggccgaaatcggcaaaatcccttataaatcaaaagaatagaccgagatagggttgagtgttgttccagtttggaacaagagtccactattaagaacgtggactccaacgtcaaagggcgaaaaaccgtctatcagggcgatggcccactacgtgaaccatcaccctaatcaagttttttggggtcgaggtgccgtaaagcactaaatcggaaccctaaagggagcccccgatttagagcttgacggggaaagccggcgaacgtggcgagaaaggaagggaagaaagcgaaaggagcgggcgctagggcgctggcaagtgtagcggtcacgctgcgcgtaaccaccacacccgccgcgcttaatgcgccgctacagggcgcgtcaggtggcacttttcggggaaatgtgcgcggaacccctatttgtttatttttctaaatacattcaaatatgtatccgctcatgagacaataaccctgataaatgcttcaataatattgaaaaaggaagagtatgagtattcaacatttccgtgtcgcc

SEQ ID NO: 10 - DNA, 11635 bp, synthetic construct
  misc_feature 1..11635: note = plasmid
  source 1..11635: mol_type = other DNA
ggtacccaactccatgcttaacagtccccaggtacagcccaccctgcgtcgcaaccaggaacagctctacagcttcctggagcgccactcgccctacttccgcagccacagtgcgcagattaggagcgccacttctttttgtcacttgaaaaacatgtaaaaataatgtactaggagacactttcaataaaggcaaatgtttttatttgtacactctcgggtgattatttaccccccacccttgccgtctgcgccgtttaaaaatcaaaggggttctgccgcgcatcgctatgcgccactggcagggacacgttgcgatactggtgtttagtgctccacttaaactcaggcacaaccatccgcggcagctcggtgaagttttcactccacaggctgcgcaccatcaccaacgcgtttagcaggtcgggcgccgatatcttgaagtcgcagttggggcctccgccctgcgcgcgcgagttgcgatacacagggttgcagcactggaacactatcagcgccgggtggtgcacgctggccagcacgctcttgtcggagatcagatccgcgtccaggtcctccgcgttgctcagggcgaacggagtcaactttggtagctgccttcccaaaaagggtgcatgcccaggctttgagttgcactcgcaccgtagtggcatcagaaggtgaccgtgcccggtctgggcgttaggatacagcgcctgcatgaaagccttgatctgcttaaaagccacctgagcctttgcgccttcagagaagaacatgccgcaagacttgccggaaaactgattggccggacaggccgcgtcatgcacgcagcaccttgcgtcggtgttggagatctgcaccacatttcggccccaccggttcttcacgatcttggccttgctagactgctccttcagcgcgcgctgcccgttttcgctcgtcacatccatttcaatcacgtgctccttatttatcataatgctcccgtgtagacacttaagctcgccttcgatctcagcgcagcggtgcagccacaacgcgcagcccgtgggctcgtggtgcttgtaggttacctctgcaaacgactgcaggtacgcctgcaggaatcgccccatcatcgtcacaaaggtcttgttgctggtgaaggtcagctgcaacccgcggtgctcctcgtttagccaggtcttgcatacggccgccagagcttccacttggtcaggcagtagcttgaagtttgcctttagatcgttatccacgtggtacttgtccatcaacgcgcgcgcagcctccatgcccttctcccacgcagacacgatcggcaggctcagcgggtttatcaccgtgctttcactttccgcttcactggactcttccttttcctcttgcgtccgcataccccgcgccactgggtcgtcttcattcagccgccgcaccgtgcgcttacctcccttgccgtgcttgattagcaccggtgggttgctgaaacccaccatttgtagcgccacatcttctctttcttcctcgctgtccacgatcacctctggggatggcgggcgctcgggcttgggagaggggcgcttctttttctttttggacgcaatggccaaatccgccgtcgaggtcgatggccgcgggctgggtgtgcgcggcaccagcgcatcttgtgacgagtcttcttcgtcctcggactcgagacgccgcctcagccgcttttttgggggcgcgcggggaggcggcggcgacggcgacggggacgacacgtcctccatggttggtggacgtcgcgccgcaccgcgtccgcgctcgggggtggtttcgcgctgctcctcttcccgactggccatttccttctcctataggcagaaaaagatcatggagtcagtcgagaaggaggacagcctaaccgccccctttgagttcgccaccaccgcctccaccgatgccgccaacgcgcctaccaccttccccgtcgaggcacccccgcttgaggaggaggaagtgattatcgagcaggacccaggttttgtaagcgaagacgacgaggatcgctcagtaccaacagaggataaaaagcaagaccaggacgacgcagaggcaaacgaggaacaagtcgggcggggggaccaaaggcatggcgactacctagatgtgggagacgacgtgctgttgaagcatctgcagcgccagtgcgccattatctgcgacgcgttgcaagagcgcagcgatgtgcccctcgccatagcggatgtcagccttgcctacgaacgccacctgttctcaccgcgcgtaccccccaaacgccaagaaaacggcacatgcgagcccaacccgcgcctcaacttctaccccgtatttgccgtgccagaggtgcttgccacctatcacatctttttccaaaactgcaagatacccctatcctgccgtgccaaccgcagccgagcggacaagcagctggccttgcggcagggcgctgtcatacctgatatcgcctcgctcgacgaagtgccaaaaatctttgagggtcttggacgcgacgagaaacgcgcggcaaacgctctgcaacaagaaaacagcgaaaatgaaagtcactgtggagtgctggtggaacttgagggtgacaacgcgcgcctagccgtgctgaaacgcagcatcgaggtcacccactttgcctacccggcacttaacctaccccccaaggttatgagcacagtcatgagcgagctgatcgtgcgccgtgcacgacccctggagagggatgcaaacttgcaagaacaaaccgaggagggcctacccgcagttggcgatgagcagctggcgcgctggcttgagacgcgcgagcctgccgacttggaggagcgacgcaagctaatgatggccgcagtgcttgttaccgtggagcttgagtgcatgcagcggttctttgctgacccggagatgcagcgcaagctagaggaaacgttgcactacacctttcgccagggctacgtgcgccaggcctgcaaaatttccaacgtggagctctgcaacctggtctcctaccttggaattttgcacgaaaaccgcctcgggcaaaacgtgcttcattccacgctcaagggcgaggcgcgccgcgactacgtccgcgactgcgtttacttatttctgtgctacacctggcaaacggccatgggcgtgtggcagcaatgcctggaggagcgcaacctaaaggagctgcagaagctgctaaagcaaaacttgaaggacctatggacggccttcaacgagcgctccgtggccgcgcacctggcggacattatcttccccgaacgcctgcttaaaaccctgcaacagggtctgccagacttcaccagtcaaagcatgttgcaaaactttaggaactttatcctagagcgttcaggaattctgcccgccacctgctgtgcgcttcctagcgactttgtgcccattaagtaccgtgaatgccctccgccgctttggggtcactgctaccttctgcagctagccaactaccttgcctaccactccgacatcatggaagacgtgagcggtgacggcctactggagtgtcactgtcgctgcaacctatgcaccccgcaccgctccctggtctgcaattcgcaactgcttagcgaaagtcaaattatcggtacctttgagctgcagggtccctcgcctgacgaaaagtccgcggctccggggttgaaactcactccggggctgtggacgtcggcttaccttcgcaaatttgtacctgaggactaccacgcccacgagattaggttctacgaagaccaatcccgcccgccaaatgcggagcttaccgcctgcgtcattacccagggccacatccttggccaattgcaagccatcaacaaagcccgccaagagtttctgctacgaaagggacggggggtttacctggacccccagtccggcgaggagctcaacccaatccccccgccgccgcagccctatcagcagccgcgggcccttgcttcccaggatggcacccaaaaagaagctgcagctgccgccgccgccacccacggacgaggaggaatactgggacagtcaggcagaggaggttttggacgaggaggaggagatgatggaagactgggacagcctagacgaagcttccgaggccgaagaggtgtcagacgaaacaccgtcaccctcggtcgcattcccctcgccggcgccccagaaattggcaaccgttcccagcatcgctacaacctccgctcctcaggcgccgccggcactgcctgttcgccgacccaaccgtagatgggacaccactggaaccagggccggtaagtctaagcagccgccgccgttagcccaagagcaacaacagcgccaaggctaccgctcgtggcgcgggcacaagaacgccatagttgcttgcttgcaagactgtgggggcaacatctccttcgcccgccgctttcttctctaccatcacggcgtggccttcccccgtaacatcctgcattactaccgtcatctctacagcccctactgcaccggcggcagcggcagcggcagcaacagcagcggtcacacagaagcaaaggcgaccggatagcaagactctgacaaagcccaagaaatccacagcggcggcagcagcaggaggaggagcgctgcgtctggcgcccaacgaacccgtatcgacccgcgagcttagaaataggatttttcccactctgtatgctatatttcaacaaagcaggggccaagaacaagagctgaaaataaaaaacaggtctctgcgctccctcacccgcagctgcctgtatcacaaaagcgaagatcagcttcggcgcacgctggaagacgcggaggctctcttcagcaaatactgcgcgctgactcttaaggactagtttcgcgccctttctcaaatttaagcgcgaaaactacgtcatctccagcggccacacccggcgccagcacctgtcgtcagcgccattatgagcaaggaaattcccacgccctacatgtggagttaccagccacaaatgggacttgcggctggagctgcccaagactactcaacccgaataaactacatgagcgcgggaccccacatgatatcccgggtcaacggaatccgcgcccaccgaaaccgaattctcctcgaacaggcggctattaccaccacacctcgtaataaccttaatccccgtagttggcccgctgccctggtgtaccaggaaagtcccgctcccaccactgtggtacttcccagagacgcccaggccgaagttcagatgactaactcaggggcgcagcttgcgggcggctttcgtcacagggtgcggtcgcccgggcgttttagggcggagtaacttgcatgtattgggaattgtagtttttttaaaatgggaagtgacgtatcgtgggaaaacggaagtgaagatttgaggaagttgtgggttttttggctttcgtttctgggcgtaggttcgcgtgcggttttctgggtgttttttgtggactttaaccgttacgtcattttttagtcctatatatactcgctctgtacttggccctttttacactgtgactgattgagctggtgccgtgtcgagtggtgttttttaataggtttttttactggtaaggctgactgttatggctgccgctgtggaagcgctgtatgttgttctggagcgggagggtgctattttgcctaggcaggagggtttttcaggtgtttatgtgtttttctctcctattaattttgttatacctcctatgggggctgtaatgttgtctctacgcctgcgggtatgtattcccccgggctatttcggtcgctttttagcactgaccgatgttaaccaacctgatgtgtttaccgagtcttacattatgactccggacatgaccgaggaactgtcggtggtgctttttaatcacggtgaccagtttttttacggtcacgccggcatggccgtagtccgtcttatgcttataagggttgtttttcctgttgtaagacaggcttctaatgtttaaatgtttttttttttgttattttattttgtgtttaatgcaggaacccgcagacatgtttgagagaaaaatggtgtctttttctgtggtggttccggaacttacctgcctttatctgcatgagcatgactacgatgtgcttgcttttttgcgcgaggctttgcctgattttttgagcagcaccttgcattttatatcgccgcccatgcaacaagcttacataggggctacgctggttagcatagctccgagtatgcgtgtcataatcagtgtgggttcttttgtcatggttcctggcggggaagtggccgcgctggtccgtgcagacctgcacgattatgttcagctggccctgcgaagggacctacgggatcgcggtatttttgttaatgttccgcttttgaatcttatacaggtctgtgaggaacctgaatttttgcaatcatgattcgctgcttgaggctgaaggtggagggcgctctggagcagatttttacaatggccggacttaatattcgggatttgcttagagacatattgataaggtggcgagatgaaaattatttgggcatggttgaaggtgctggaatgtttatagaggagattcaccctgaagggtttagcctttacgtccacttggacgtgagggcagtttgccttttggaagccattgtgcaacatcttacaaatgccattatctgttctttggctgtagagtttgaccacgccaccggaggggagcgcgttcacttaatagatcttcattttgaggttttggataatcttttggaataaaaaaaaaaaaacatggttcttccagctcttcccgctcctcccgtgtgtgactcgcagaacgaatgtgtaggttggctgggtgtggcttattctgcggtggtggatgttatcagggcagcggcgcatgaaggagtttacatagaacccgaagccagggggcgcctggatgctttgagagagtggatatactacaactactacacagagcgagctaagcgacgagaccggagacgcagatctgtttgtcacgcccgcacctggttttgcttcaggaaatatgactacgtccggcgttccatttggcatgacactacgaccaacacgatctcggttgtctcggcgcactccgtacagtagggatcgcctacctccttttgagacagagacccgcgctaccatactggaggatcatccgctgctgcccgaatgtaacactttgacaatgcacaacgtgagttacgtgcgaggtcttccctgcagtgtgggatttacgctgattcaggaatgggttgttccctgggatatggttctgacgcgggaggagcttgtaatcctgaggaagtgtatgcacgtgtgcctgtgttgtgccaacattgatatcatgacgagcatgatgatccatggttacgagtcctgggctctccactgtcattgttccagtcccggttccctgcagtgcatagccggcgggcaggttttggccagctggtttaggatggtggtggatggcgccatgtttaatcagaggtttatatggtaccgggaggtggtgaattacaacatgccaaaagaggtaatgtttatgtccagcgtgtttatgaggggtcgccacttaatctacctgcgcttgtggtatgatggccacgtgggttctgtggtccccgccatgagctttggatacagcgccttgcactgtgggattttgaacaatattgtggtgctgtgctgcagttactgtgctgatttaagtgagatcagggtgcgctgctgtgcccggaggacaaggcgtctcatgctgcgggcggtgcgaatcatcgctgaggagaccactgccatgttgtattcctgcaggacggagcggcggcggcagcagtttattcgcgcgctgctgcagcaccaccgccctatcctgatgcacgattatgactctacccccatgtaggcgtggacttccccttcgccgcccgttgagcaaccgcaagttggacagcagcctgtggctcagcagctggacagcgacatgaacttaagcgagctgcccggggagtttattaatatcactgatgagcgtttggctcgacaggaaaccgtgtggaatataacacctaagaatatgtctgttacccatgatatgatgctttttaaggccagccggggagaaaggactgtgtactctgtgtgttgggagggaggtggcaggttgaatactagggttctgtgagtttgattaaggtacggtgatcaatataagctatgtggtggtggggctatactactgaatgaaaaatgacttgaaattttctgcaattgaaaaataaacacgttgaaacataacatgcaacaggttcacgattctttattcctgggcaatgtaggagaaggtgtaagagttggtagcaaaagtttcagtggtgtattttccactttcccaggaccatgtaaaagacatagagtaagtgcttacctcgctagtttctgtggattcactagaatcgatgtaggatgttgcccctcctgacgcggtaggagaaggggagggtgccctgcatgtctgccgctgctcttgctcttgccgctgctgaggaggggggcgcatctgccgcagcaccggatgcatctgggaaaagcaaaaaaggggctcgtccctgtttccggaggaatttgcaagcggggtcttgcatgacggggaggcaaacccccgttcgccgcagtccggccggcccgagactcgaaccgggggtcctgcgactcaacccttggaaaataaccctccggctacagggagcgagccacttaatgctttcgctttccagcctaaccgcttacgccgcgcgcggccagtggccaaaaaagctagcgcagcagccgccgcgcctggaaggaagccaaaaggagcgctcccccgttgtctgacgtcgcacacctgggttcgacacgcgggcggtaaccgcatggatcacggcggacggccggatccggggttcgaaccccggtcgtccgccatgatacccttgcgaatttatccaccagaccacggaagagtgcccgcttacaggctctccttttgcacggtctagagcgtcaacgactgcgcacgcctcaccggccagagcgtcccgaccatggagcactttttgccgctgcgcaacatctggaaccgcgtccgcgactttccgcgcgcctccaccaccgccgccggcatcacctggatgtccaggtacatctacggattacgtcgacgtttaaaccatatgatcagctcactcaaaggcggtaatacggttatccacagaatcaggggataacgcaggaaagaacatgtgagcaaaaggccagcaaaaggccaggaaccgtaaaaaggccgcgttgctggcgtttttccataggctccgcccccctgacgagcatcacaaaaatcgacgctcaagtcagaggtggcgaaacccgacaggactataaagataccaggcgtttccccctggaagctccctcgtgcgctctcctgttccgaccctgccgcttaccggatacctgtccgcctttctcccttcgggaagcgtggcgctttctcatagctcacgctgtaggtatctcagttcggtgtaggtcgttcgctccaagctgggctgtgtgcacgaaccccccgttcagcccgaccgctgcgccttatccggtaactatcgtcttgagtccaacccggtaagacacgacttatcgccactggcagcagccactggtaacaggattagcagagcgaggtatgtaggcggtgctacagagttcttgaagtggtggcctaactacggctacactagaagaacagtatttggtatctgcgctctgctgaagccagttaccttcggaaaaagagttggtagctcttgatccggcaaacaaaccaccgctggtagcggtggtttttttgtttgcaagcagcagattacgcgcagaaaaaaaggatctcaagaagatcctttgatcttttctacggggtctgacgctcagtggaacgaaaactcacgttaagggattttggtcatgagattatcaaaaaggatcttcacctagatccttttaaattaaaaatgaagttttaaatcaatctaaagtatatatgagtaaacttggtctgacagttaccaatgcttaatcagtgaggcacctatctcagcgatctgtctatttcgttcatccatagttgcctgactccccgtcgtgtagataactacgatacgggagggcttaccatctggccccagtgctgcaatgataccgcgagacccacgctcaccggctccagatttatcagcaataaaccagccagccggaagggccgagcgcagaagtggtcctgcaactttatccgcctccatccagtctattaattgttgccgggaagctagagtaagtagttcgccagttaatagtttgcgcaacgttgttgccattgctacaggcatcgtggtgtcacgctcgtcgtttggtatggcttcattcagctccggttcccaacgatcaaggcgagttacatgatcccccatgttgtgcaaaaaagcggttagctccttcggtcctccgatcgttgtcagaagtaagttggccgcagtgttatcactcatggttatggcagcactgcataattctcttactgtcatgccatccgtaagatgcttttctgtgactggtgagtactcaaccaagtcattctgagaatagtgtatgcggcgaccgagttgctcttgcccggcgtcaatacgggataataccgcgccacatagcagaactttaaaagtgctcatcattggaaaacgttcttcggggcgaaaactctcaaggatcttaccgctgttgagatccagttcgatgtaacccactcgtgcacccaactgatcttcagcatcttttactttcaccagcgtttctgggtgagcaaaaacaggaaggcaaaatgccgcaaaaaagggaataagggcgacacggaaatgttgaatactcatactcttcctttttcaatattattgaagcatttatcagggttattgtctcatgagcggatacatatttgaatgtatttagaaaaataaacaaataggggttccgcgcacatttccccgaaaagtgccacctaaattgtaagcgttaatattttgttaaaattcgcgttaaatttttgttaaatcagctcattttttaaccaataggccgaaatcggcaaaatcccttataaatcaaaagaatagaccgagatagggttgagtgttgttccagtttggaacaagagtccactattaaagaacgtggactccaacgtcaaagggcgaaaaaccgtctatcagggcgatggcccactacgtgaaccatcaccctaatcaagttttttggggtcgaggtgccgtaaagcactaaatcggaaccctaaagggagcccccgatttagagcttgacggggaaagccggcgaacgtggcgagaaaggaagggaagaaagcgaaaggagcgggcgctagggcgctggcaagtgtagcggtcacgctgcgcgtaaccaccacacccgccgcgcttaatgcgccgctacagggcgcgatggatcc